European Patent Application EP 4 667 497 A1, published December 24, 2025. Title: BISPECIFIC ANTIBODY AND USE THEREOF. Applicant: Shaoxing Institute, Zhejiang University. The sequence listing filed with the application follows.

SEQUENCE LISTING (108 sequences)

SEQ ID NO: 1 - protein, 80 aa, synthetic construct
VTCKSGDFSCGGRVNRCIPQFWRCDGQVDCDNGSDEQGCPPKTCSQDEFRCHDGKCISRQFVCDSDRDCLDGSDEASCPV

SEQ ID NO: 2 - protein, 553 aa, synthetic construct
MDWTWRILFLVAAATGAHSQVQLQQSGAELARPGASVKMSCKASGYTFTRYTMHWVKQRPGQGLEWIGYINPSRGYTNYNQKFKDKATLTTDKSSSTAYMQLSSLTSEDSAVYYCARYYDDHYCLDYWGQGTTLTVSSASTKGPSVFPLAPSSKSTSGGTAALGCLVKDYFPEPVTVSWNSGALTSGVHTFPAVLQSSGLYSLSSVVTVPSSSLGTQTYICNVNHKPSNTKVDKKVEPKSCDKTHTCPPCPAPELLGGPSVFLFPPKPKDTLMISRTPEVTCVVVDVSHEDPEVKFNWYVDGVEVHNAKTKPREEQYNSTYRVVSVLTVLHQDWLNGKEYKCKVSNKALPAPIEKTISKAKGQPREPQVYTLPPSRDELTKNQVSLTCLVKGFYPSDIAVEWESNGQPENNYKTTPPVLDSDGSFFLYSKLTVDKSRWQQGNVFSCSVMHEALHNHYTQKSLSLSPGKGGGGSVTCKSGDFSCGGRVNRCIPQFWRCDGQVDCDNGSDEQGCPPKTCSQDEFRCHDGKCISRQFVCDSDRDCLDGSDEASCPV

SEQ ID NO: 3 - protein, 234 aa, synthetic construct
METDTLLLWVLLLWVPGSTGQIVLTQSPAIMSASPGEKVTMTCSASSSVSYMNWYQQKSGTSPKRWIYDTSKLASGVPAHFRGSGSGTSYSLTISGMEAEDAATYYCQQWSSNPFTFGSGTKLEINRRTVAAPSVFIFPPSDEQLKSGTASVVCLLNNFYPREAKVQWKVDNALQSGNSQESVTEQDSKDSTYSLSSTLTLSKADYEKHKVYACEVTHQGLSSPVTKSFNRGEC

SEQ ID NO: 4 - protein, 557 aa, synthetic construct
MDWTWRILFLVAAATGAHSQVQLVESGGGLVQPGGSLKLSCAASGFDFSRYWMSWVRQAPGKGLEWIGEINPTSSTINFTPSLKDKVFISRDNAKNTLYLQMSKVRSEDTALYYCARGNYYRYGDAMDYWGQGTSVTVSKISASTKGPSVFPLAPSSKSTSGGTAALGCLVKDYFPEPVTVSWNSGALTSGVHTFPAVLQSSGLYSLSSVVTVPSSSLGTQTYICNVNHKPSNTKVDKKVEPKSCDKTHTCPPCPAPELLGGPSVFLFPPKPKDTLMISRTPEVTCVVVDVSHEDPEVKFNWYVDGVEVHNAKTKPREEQYNSTYRVVSVLTVLHQDWLNGKEYKCKVSNKALPAPIEKTISKAKGQPREPQVYTLPPSRDELTKNQVSLTCLVKGFYPSDIAVEWESNGQPENNYKTTPPVLDSDGSFFLYSKLTVDKSRWQQGNVFSCSVMHEALHNHYTQKSLSLSPGKGGGGSVTCKSGDFSCGGRVNRCIPQFWRCDGQVDCDNGSDEQGCPPKTCSQDEFRCHDGKCISRQFVCDSDRDCLDGSDEASCPV

SEQ ID NO: 5 - protein, 239 aa, synthetic construct
METDTLLLWVLLLWVPGSTGSDIVLTQSPASLAVSLGQRATISCRASKSVSTSGYSYLHWYQQKPGQPPKLLIYLASNLESGVPARFSGSGSGTDFTLNIHPVEEEDAATYYCQHSRELPFTFGSGTKLEIKRTVAAPSVFIFPPSDEQLKSGTASVVCLLNNFYPREAKVQWKVDNALQSGNSQESVTEQDSKDSTYSLSSTLTLSKADYEKHKVYACEVTHQGLSSPVTKSFNRGEC

SEQ ID NO: 6 - protein, 577 aa, synthetic construct
MGWSCIILFLVATATGVHSDIQMTQTTSSLSASLGDRVTISCRASQDISKYLNWYQQKPDGTVKLLIYHTSRLHSGVPSRFSGSGSGTDYSLTISNLEQEDIATYFCQQGNTLPYTFGGGTKLEITGGGGSGGGGSGGGGSEVKLQESGPGLVAPSQSLSVTCTVSGVSLPDYGVSWIRQPPRKGLEWLGVIWGSETTYYNSALKSRLTIIKDNSKSQVFLKMNSLQTDDTAIYYCAKHYYYGGSYAMDYWGQGTSVTVSSPKSCDKTHTCPPCPAPELLGGPSVFLFPPKPKDTLMISRTPEVTCVVVDVSHEDPEVKFNWYVDGVEVHNAKTKPREEQYNSTYRVVSVLTVLHQDWLNGKEYKCKVSNKALPAPIEKTISKAKGQPREPQVYTLPPSRDELTKNQVSLTCLVKGFYPSDIAVEWESNGQPENNYKTTPPVLDSDGSFFLYSKLTVDKSRWQQGNVFSCSVMHEALHNHYTQKSLSLSPGKGGGGSVTCKSGDFSCGGRVNRCIPQFWRCDGQVDCDNGSDEQGCPPKTCSQDEFRCHDGKCISRQFVCDSDRDCLDGSDEASCPV

SEQ ID NO: 7 - protein, 30 aa, synthetic construct
  VARIANT 6..30: note = Up to 5 copies of GGGGS can be deleted; note (original language) = 最多可删除5个GGGGS序列
GGGGSGGGGSGGGGSGGGGSGGGGSGGGGS

SEQ ID NO: 8 - protein, 31 aa, synthetic construct
  VARIANT 6..30: note = Up to 5 copies of GGGGS can be deleted; note (original language) = 最多可删除5个GGGGS序列
GGGGSGGGGSGGGGSGGGGSGGGGSGGGGSA

SEQ ID NO: 9 - protein, 15 aa, synthetic construct
EPKSSDKTHTCPPCP

SEQ ID NO: 10 - protein, 10 aa, synthetic construct
DKTHTCPPCP

SEQ ID NO: 11 - protein, 5 aa, synthetic construct
GGGGS

SEQ ID NO: 12 - protein, 15 aa, synthetic construct
GGGGSGGGGSGGGGS

SEQ ID NO: 13 - protein, 16 aa, synthetic construct
GGGGSGGGGSGGGGSA

SEQ ID NO: 14 - protein, 21 aa, synthetic construct
GGGGSGGGGSGGGGSGGGGSA

SEQ ID NO: 15 - DNA, 38 bp, synthetic construct
  source 1..38: mol_type = other DNA
gcaaccggtgtacattctgatatacagatgacgcagac

SEQ ID NO: 16 - DNA, 36 bp, synthetic construct
  source 1..36: mol_type = other DNA
gtcgcagctcttgggtgaactcactgtcactgacgt

SEQ ID NO: 17 - DNA, 23 bp, synthetic construct
  source 1..23: mol_type = other DNA
cccaagagctgcgacaagaccca

SEQ ID NO: 18 - DNA, 33 bp, synthetic construct
  source 1..33: mol_type = other DNA
agatcctccgccgcctttgccaggagacaggct

SEQ ID NO: 19 - DNA, 32 bp, synthetic construct
  source 1..32: mol_type = other DNA
ggcggcggaggatctgtgacctgcaagtccgg

SEQ ID NO: 20 - DNA, 35 bp, synthetic construct
  source 1..35: mol_type = other DNA
cggccgtcgcactcacacaggacagctggcctcgt

SEQ ID NO: 21 - DNA, 35 bp, synthetic construct
  source 1..35: mol_type = other DNA
acaggtgcccattctcaagtgcagctccagcagag

SEQ ID NO: 22 - DNA, 35 bp, synthetic construct
  source 1..35: mol_type = other DNA
acccttggtgctggcagaggacacggtcagggttg

SEQ ID NO: 23 - DNA, 20 bp, synthetic construct
  source 1..20: mol_type = other DNA
gccagcaccaagggtcccag

SEQ ID NO: 24 - DNA, 35 bp, synthetic construct
  source 1..35: mol_type = other DNA
agatcctccgccgccctttccggggctcaggctca

SEQ ID NO: 25 - DNA, 32 bp, synthetic construct; identical to SEQ ID NO: 19
  source 1..32: mol_type = other DNA

SEQ ID NO: 26 - DNA, 38 bp, synthetic construct
  source 1..38: mol_type = other DNA
gatcgaaccctttcatcacacaggacagctggcctcgt

SEQ ID NO: 27 - DNA, 35 bp, synthetic construct
  source 1..35: mol_type = other DNA
ccaggctctaccggccaaatcgtgctgacacagag

SEQ ID NO: 28 - DNA, 35 bp, synthetic construct
  source 1..35: mol_type = other DNA
ggcagccacggtccttctgttgatttccagcttgg

SEQ ID NO: 29 - DNA, 20 bp, synthetic construct
  source 1..20: mol_type = other DNA
aggaccgtggctgcccccag

SEQ ID NO: 30 - DNA, 38 bp, synthetic construct
  source 1..38: mol_type = other DNA
gatcgaaccctttcatcagcactcgcccctgttgaagc

SEQ ID NO: 31 - DNA, 35 bp, synthetic construct
  source 1..35: mol_type = other DNA
acaggtgcccattctcaagtgcaactggtggaatc

SEQ ID NO: 32 - DNA, 35 bp, synthetic construct
  source 1..35: mol_type = other DNA
acccttggtgctggcgctgattttggacactgtca

SEQ ID NO: 33 - DNA, 35 bp, synthetic construct
  source 1..35: mol_type = other DNA
ccaggctctaccggcagcgacatcgtgctgaccca

SEQ ID NO: 34 - DNA, 35 bp, synthetic construct
  source 1..35: mol_type = other DNA
ggcagccacggtcctcttgatctcgagcttggtgc

SEQ ID NO: 35 - DNA, 35 bp, synthetic construct
  source 1..35: mol_type = other DNA
acaggtgcccattctgaggtgcagctgcagcaaag

SEQ ID NO: 36 - DNA, 35 bp, synthetic construct
  source 1..35: mol_type = other DNA
acccttggtgctggcgctgaacacggtcagggtgg

SEQ ID NO: 37 - DNA, 35 bp, synthetic construct
  source 1..35: mol_type = other DNA
ccaggctctaccggcatggacattcagatgaccca

SEQ ID NO: 38 - DNA, 36 bp, synthetic construct
  source 1..36: mol_type = other DNA
ggcagccacggtcctcttgatttccagctttgttcc

SEQ ID NO: 39 - DNA, 35 bp, synthetic construct
  source 1..35: mol_type = other DNA
acaggtgcccattctgaggtgcaactggtggaaag

SEQ ID NO: 40 - DNA, 35 bp, synthetic construct
  source 1..35: mol_type = other DNA
acccttggtgctggcggaggacactgtaaccagga

SEQ ID NO: 41 - DNA, 36 bp, synthetic construct
  source 1..36: mol_type = other DNA
ccaggctctaccggcgatatccagctgacacagtct

SEQ ID NO: 42 - DNA, 35 bp, synthetic construct
  source 1..35: mol_type = other DNA
ggcagccacggtcctcttgatttccagcttggtgc

SEQ ID NO: 43 - DNA, 39 bp, synthetic construct
  source 1..39: mol_type = other DNA
acaggtgcccattctcaagtgcagctgcagcagccagga

SEQ ID NO: 44 - DNA, 35 bp, synthetic construct
  source 1..35: mol_type = other DNA
acccttggtgctggcggcggacacggtcacggttg

SEQ ID NO: 45 - DNA, 35 bp, synthetic construct
  source 1..35: mol_type = other DNA
ccaggctctaccggccaaatcgtgctgtctcagag

SEQ ID NO: 46 - DNA, 36 bp, synthetic construct
  source 1..36: mol_type = other DNA
ggcagccacggtcctcttaatttccagctttgttcc

SEQ ID NO: 47 - DNA, 35 bp, synthetic construct
  source 1..35: mol_type = other DNA
acaggtgcccattctcaagtgcagctggtcgagag

SEQ ID NO: 48 - DNA, 35 bp, synthetic construct
  source 1..35: mol_type = other DNA
acccttggtgctggcggaggacacggtcaccagtg

SEQ ID NO: 49 - DNA, 38 bp, synthetic construct
  source 1..38: mol_type = other DNA
ccaggctctaccggcatggacatgcgggtccccgccca

SEQ ID NO: 50 - DNA, 36 bp, synthetic construct
  source 1..36: mol_type = other DNA
ggcagccacggtccttttgatttccaccttggttcc

SEQ ID NO: 51 - DNA, 35 bp, synthetic construct
  source 1..35: mol_type = other DNA
acaggtgcccattctcaggtgcagctgaaacagag

SEQ ID NO: 52 - DNA, 36 bp, synthetic construct
  source 1..36: mol_type = other DNA
acccttggtgctggcagcagacacggtcaccagggt

SEQ ID NO: 53 - DNA, 39 bp, synthetic construct
  source 1..39: mol_type = other DNA
ccaggctctaccggctctatcgtgatgacccaaacacct

SEQ ID NO: 54 - DNA, 39 bp, synthetic construct
  source 1..39: mol_type = other DNA
ggcagccacggtccttctgatttccagctttgtgcctcc

SEQ ID NO: 55 - DNA, 4808 bp, synthetic construct
  source 1..4808: mol_type = other DNA
cccatatatggagttccgcgttacataacttacggtaaatggcccgcctggctgaccgcccaacgacccccgcccatgacgtcaataatgacgtatgttcccatagtaacgccaatagggactttccattgacgtcaatgggtggagtatttacggtaaactgcccacttggcagtacatcaagtgtatcatatgccaagtacgccccctattgacgtcaatgacggtaaatggcccgcctggcattatgcccagtacatgaccttatgggactttcctacttggcagtacatctacgtattagtcatcgctattaccatggtgatgcggttttggcagtacatcaatgggcgtggatagcggtttgactcacggggatttccaagtctccaccccattgacgtcaatgggagtttgttttggcaccaaaatcaacgggactttccaaaatgtcgtaacaactccgccccattgacgcaaatgggcggtaggcgtgtacggtgggaggtctatataagcagagctcgtttagtgaaccgtcagatcgcctggagacgccatccacgctgttttgacctccatagaagacaccgggaccgatccagcctccgcggccgggaacggtgcattggaacgcggattccccgtgccaagagtgacgtaagtaccgcctatagagtctataggcccacccccttggcttcgttagaacgcggctacaattaatacataaccttatgtatcatacacatacgatttaggtgacactatagaataacatccactttgcctttctctccacaggtgtccactcccaggtccaactgcacctcggttctatcgattgaattccaccatgggatggtcatgtatcatcctttttctagtagcaactgcaaccggtgtacattctggagaccttattagagctcatactccatatattaattttacaattgtgaacggtctcatgagtgcgacggccggcaagcccccgctccccgggctctcgcggtcgtacgaggaaagcttggccgccatggcccaacttgtttattgcagcttataatggttacaaataaagcaatagcatcacaaatttcacaaataaagcatttttttcactgcattctagttgtggtttgtccaaactcatcaatgtatcttatcatgtctggatcgggaattaattcggcgcagcaccatggcctgaaataacctctgaaagaggaacttggttaggtaccttctgaggcggaaagaaccatctgtggaatgtgtgtcagttagggtgtggaaagtccccaggctccccagcaggcagaagtatgcaaagcatgcatctcaattagtcagcaaccaggtgtggaaagtccccaggctccccagcaggcagaagtatgcaaagcatgcatctcaattagtcagcaaccatagtcccgcccctaactccgcccatcccgcccctaactccgcccagttccgcccattctccgccccatggctgactaattttttttatttatgcagaggccgaggccgcctcggcctctgagctattccagaagtagtgaggaggcttttttggaggcctaggcttttgcaaammgckgktamcagctygrcactggccgtcgttttacaacgtcgtgactgggaaaaccctggcgttacccaacttaatcgccttgcagcacatccccctttcgccagytggcgtaatagcgaagaggcccgcaccgatcgcccttcccaacagttgcgcagcctgaatggcgaatggcgcctgatgcggtattttctccttacgcatctgtgcggtatttcacaccgcatacgtsrwagcamycwyagtacratctgcyctgtakcgscgcattaagcgcggcgggtgtggtggttacgcgcagcgtgaccgctacacttgccagcgccctagcgcccgctcctttcgctttcttcccttcctttctcgccacgttcgccggctttccccgtcaagctctaaatcgggggctccctttagggttccgatttagtgctttacggcacctcgaccccaaaaaacttgatttgggtgatggttcacgtagtgggccatcgccctgatagacggtttttcgccctttgacgttggagtccacgttctttaatagtggactcttgttccaaactggaacaacactcaaccctatctcgggctattcttttgatttataagggattttgccgatttcggcctattggttaaaaaatgagctgatttaacaaaaatttaacgcgaattttaacaaaatattaacgtttacaattttatggtgcactctcagtacaatctgctctgatgccgcatagttaagccagccccgacacccgccaacacccgctgacgcgccctgacgggcttgtctgctcccggcatccgcttacagacaagctgtgaccgtctccgggagctgcatgtgtcagaggttttcaccgtcatcaccgaaacgcgcgagacgaaagggcctcgtgatacgcctatttttataggttaatgtcatgataataatggtttcttagacgtcaggtggcacttttcggggaaatgtgcgcggaacccctatttgtttatttttctaaatacattcaaatatgtatccgctcatgagacaataaccctgataaatgcttcaataatattgaaaaaggaagagtatgagtattcaacatttccgtgtcgcccttattcccttttttgcggcattttgccttcctgtttttgctcacccagaaacgctggtgaaagtaaaagatgctgaagatcagttgggtgcacgagtgggttacatcgaactggatctcaacagcggtaagatccttgagagttttcgccccgaagaacgttttccaatgatgagcacttttaaagttctgctatgtggcgcggtattatcccgtattgacgccgggcaagagcaactcggtcgccgcatacactattctcagaatgacttggttgagtactcaccagtcacagaaaagcatcttacggatggcatgacagtaagagaattatgcagtgctgccataaccatgagtgataacactgcggccaacttacttctgacaacgatcggaggaccgaaggagctaaccgcttttttgcacaacatgggggatcatgtaactcgccttgatcgttgggaaccggagctgaatgaagccataccaaacgacgagcgtgacaccacgatgcctgtagcaatggcaacaacgttgcgcaaactattaactggcgaactacttactctagcttcccggcaacaattaatagactggatggaggcggataaagttgcaggaccacttctgcgctcggcccttccggctggctggtttattgctgataaatctggagccggtgagcgtgggtctcgcggtatcattgcagcactggggccagatggtaagccctcccgtatcgtagttatctacacgacggggagtcaggcaactatggatgaacgaaatagacagatcgctgagataggtgcctcactgattaagcattggtaactgtcagaccaagtttactcatatatactttagattgatttaaaacttcatttttaatttaaaaggatctaggtgaagatcctttttgataatctcatgaccaaaatcccttaacgtgagttttcgttccactgagcgtcagaccccgtagaaaagatcaaaggatcttcttgagatcctttttttctgcgcgtaatctgctgcttgcaaacaaaaaaaccaccgctaccagcggtggtttgtttgccggatcaagagctaccaactctttttccgaaggtaactggcttcagcagagcgcagataccaaatactgttcttctagtgtagccgtagttaggccaccacttcaagaactctgtagcaccgcctacatacctcgctctgctaatcctgttaccagtggctgctgccagtggcgataagtcgtgtcttaccgggttggactcaagacgatagttaccggataaggcgcagcggtcgggctgaacggggggttcgtgcacacagcccagcttggagcgaacgacctacaccgaactgagatacctacagcgtgagctatgagaaagcgccacgcttcccgaagggagaaaggcggacaggtatccggtaagcggcagggtcggaacaggagagcgcacgagggagcttccagggggaaacgcctggtatctttatagtcctgtcgggtttcgccacctctgacttgagcgtcgatttttgtgatgctcgtcaggggggcggagcctatggaaaaacgccagcaacgcggcctttttacggttcctggccttttgctggccttttgctcacatgttctttcctgcgttatcccctgattctgtggataaccgtattaccgcctttgagtgagctgataccgctcgccgcagccgaacgaccgagcgcagcgagtcagtgagcgaggaagcggaagagcgcccaatacgcaaaccgcctctccccgcgcgttggccgattcattaatccaactggcacgacaggtttcccgactggaaagcgggcagtgagcgcaacgcaattaatgtgagttagctcactcattaggcaccccaggctttacactttatgcttccggctcgtatgttgtgtggaattgtgagcggataacaatttcacacaggaaacagctatgacatgattacgaattaattcgagctcgcccgacattgattattgactagttattaatagtaatcaattacggggtcattagttcatag

SEQ ID NO: 56 - DNA, 726 bp, synthetic construct
  source 1..726: mol_type = other DNA
gatatacagatgacgcagacaacgtcaagtctttccgccagcttgggagaccgagtgactatatcttgtagagcaagccaggatatttctaagtatcttaactggtaccaacaaaagcccgatggaacggttaagctgcttatataccataccagtagactccactccggcgtaccatcacggttttctggcagtggctccgggaccgactattctttgacgatctctaatctcgaacaagaggatattgcaacatacttttgtcagcaaggcaataccttgccatatacgtttgggggcgggacaaaacttgagataaccggcggcggtggttcaggcggtggcggttccggtggtgggggatcagaggttaagcttcaggaatccggaccaggtttggttgcccccagccaatctctcagcgttacatgcacggtttcaggcgtcagtctccccgattacggtgtaagttggattcggcaacctccgcgaaagggtctggaatggctgggggttatttgggggagtgagacaacttattacaactctgcacttaagagtcggcttaccatcatcaaggataattcaaaatcacaagtattcctgaagatgaactcattgcaaacagatgatacagctatatactattgtgccaagcattactattatggtggttcttatgcaatggattactgggggcaaggcacgtcagtgacagtgagttca

SEQ ID NO: 57 - DNA, 693 bp, synthetic construct
  source 1..693: mol_type = other DNA
cccaagagctgcgacaagacccacacctgtcctccatgtcctgctccagaactgctcggcggaccttccgtgttcctgtttcctccaaagcctaaggacaccctgatgatcagcagaacccctgaagtgacctgcgtggtggtggatgtgtcccacgaggatcccgaagtgaagttcaattggtacgtggacggcgtggaagtgcacaacgccaagaccaagcctagagaggaacagtacaacagcacctacagagtggtgtccgtgctgaccgtgctgcaccaggattggctgaacggcaaagagtacaagtgcaaggtgtccaacaaggccctgcctgctcctatcgagaaaaccatcagcaaggccaagggccagcctagggaaccccaggtttacacactgcctccaagcagggacgagctgaccaagaatcaggtgtccctgacctgcctggtcaagggcttctacccttccgatatcgccgtggaatgggagagcaatggccagcctgagaacaactacaagacaacccctcctgtgctggacagcgacggctcattcttcctgtacagcaagctgacagtggacaagagcagatggcagcagggcaacgtgttcagctgcagcgtgatgcacgaggccctgcacaaccactacacccagaagtccctgagcctgtctcctggcaaa

SEQ ID NO: 58 - DNA, 240 bp, synthetic construct
  source 1..240: mol_type = other DNA
gtgacctgcaagtccggcgacttcagctgcggcggaagagtgaatagatgcatcccccaattttggcggtgtgatggccaggtcgactgcgacaacggctctgatgaacagggctgtcctcctaagacatgttctcaggacgagttcagatgccacgacggcaaatgcatcagcagacagttcgtgtgcgacagcgatagagattgcctcgacggctccgacgaggccagctgtcctgtg

SEQ ID NO: 59 - DNA, 6138 bp, synthetic construct
  source 1..6138: mol_type = other DNA
gttaggcgttttgcgctgcttcgcgatgtacgggccagatatacgcgttgacattgattattgactagttattaatagtaatcaattacggggtcattagttcatagcccatatatggagttccgcgttacataacttacggtaaatggcccgcctggctgaccgcccaacgacccccgcccattgacgtcaataatgacgtatgttcccatagtaacgccaatagggactttccattgacgtcaatgggtggagtatttacggtaaactgcccacttggcagtacatcaagtgtatcatatgccaagtacgccccctattgacgtcaatgacggtaaatggcccgcctggcattatgcccagtacatgaccttatgggactttcctacttggcagtacatctacgtattagtcatcgctattaccatggtgatgcggttttggcagtacatcaatgggcgtggatagcggtttgactcacggggatttccaagtctccaccccattgacgtcaatgggagtttgttttggcaccaaaatcaacgggactttccaaaatgtcgtaacaactccgccccattgacgcaaatgggcggtaggcgtgtacggtgggaggtctatataagcagagctcgtttagtgaaccgtcagatcgcctggagacgccatccacgctgttttgacctccatagaagacaccgggaccgatccagcctccggactctagaggatcgaacccttgccaccatggactggacatggcggatcctgtttctggtggctgctgccacaggtgcccattctggagaccttattagagctcatactccatatattaattttacaattgtgaacggtctcatgatgaaagggttcgatccctaccggttagtaatgagtttgatatctcgacaatcaacctctggattacaaaatttgtgaaagattgactggtattcttaactatgttgctccttttacgctatgtggatacgctgctttaatgcctttgtatcatgctattgcttcccgtatggctttcattttctcctccttgtataaatcctggttgctgtctctttatgaggagttgtggcccgttgtcaggcaacgtggcgtggtgtgcactgtgtttgctgacgcaacccccactggttggggcattgccaccacctgtcagctcctttccgggactttcgctttccccctccctattgccacggcggaactcatcgccgcctgccttgcccgctgctggacaggggctcggctgttgggcactgacaattccgtggtgttgtcggggaagctgacgtcctttccatggctgctcgcctgtgttgccacctggattctgcgcgggacgtccttctgctacgtcccttcggccctcaatccagcggaccttccttcccgcggcctgctgccggctctgcggcctcttccgcgtcttcgccttcgccctcagacgagtcggatctccctttgggccgcctccccgcctggaaacgggggaggctaactgaaacacggaaggagacaataccggaaggaacccgcgctatgacggcaataaaaagacagaataaaacgcacgggtgttgggtcgtttgttcataaacgcggggttcggtcccagggctggcactctgtcgataccccaccgtgaccccattggggccaatacgcccgcgtttcttccttttccccaccccaccccccaagttcgggtgaaggcccagggctcgcagccaacgtcggggcggcaggccctgccatagcagatctgcgcagctggggctctagggggtatccccacgcgccctgtagcggcgcattaagcgcggcgggtgtggtggttacgcgcagcgtgaccgctacacttgccagcgccctagcgcccgctcctttcgctttcttcccttcctttctcgccacgttcgccggctttccccgtcaagctctaaatcggggcatccctttagggttccgatttagtgctttacggcacctcgaccccaaaaaacttgattagggtgatggttcacgtagtgggccatcgccctgatagacggtttttcgccctttgacgttggagtccacgttctttaatagtggactcttgttccaaactggaacaacactcaaccctatctcggtctattcttttgatttataagggattttggggatttcggcctattggttaaaaaatgagctgatttaacaaaaatttaacgcgaattaattctgtggaatgtgtgtcagttagggtgtggaaagtccccaggctccccagcaggcagaagtatgcaaagcatgcatctcaattagtcagcaaccaggtgtggaaagtccccaggctccccagcaggcagaagtatgcaaagcatgcatctcaattagtcagcaaccatagtcccgcccctaactccgcccatcccgcccctaactccgcccagttccgcccattctccgccccatggctgactaattttttttatttatgcagaggccgaggccgcctctgcctctgagctattccagaagtagtgaggaggcttttttggaggcctaggcttttgcaaaaagctcccgggagcttgtatatccattttcggatctgatcaagagacaggatgaggatcgtttcgcatgattgaacaagatggattgcacgcaggttctccggccgcttgggtggagaggctattcggctatgactgggcacaacagacaatcggctgctctgatgccgccgtgttccggctgtcagcgcaggggcgcccggttctttttgtcaagaccgacctgtccggtgccctgaatgaactgcaggacgaggcagcgcggctatcgtggctggccacgacgggcgttccttgcgcagctgtgctcgacgttgtcactgaagcgggaagggactggctgctattgggcgaagtgccggggcaggatctcctgtcatctcaccttgctcctgccgagaaagtatccatcatggctgatgcaatgcggcggctgcatacgcttgatccggctacctgcccattcgaccaccaagcgaaacatcgcatcgagcgagcacgtactcggatggaagccggtcttgtcgatcaggatgatctggacgaagagcatcaggggctcgcgccagccgaactgttcgccaggctcaaggcgcgcatgcccgacggcgaggatctcgtcgtgacccatggcgatgcctgcttgccgaatatcatggtggaaaatggccgcttttctggattcatcgactgtggccggctgggtgtggcggaccgctatcaggacatagcgttggctacccgtgatattgctgaagagcttggcggcgaatgggctgaccgcttcctcgtgctttacggtatcgccgctcccgattcgcagcgcatcgccttctatcgccttcttgacgagttcttctgagcgggactctggggttcgcgaaatgaccgaccaagcgacgcccaacctgccatcacgagatttcgattccaccgccgccttctatgaaaggttgggcttcggaatcgttttccgggacgccggctggatgatcctccagcgcggggatctcatgctggagttcttcgcccaccccaacttgtttattgcagcttataatggttacaaataaagcaatagcatcacaaatttcacaaataaagcatttttttcactgcattctagttgtggtttgtccaaactcatcaatgtatcttatcatgtctgtataccgtcgacctctagctagagcttggcgtaatcatggtcatagctgtttcctgtgtgaaattgttatccgctcacaattccacacaacatacgagccggaagcataaagtgtaaagcctggggtgcctaatgagtgagctaactcacattaattgcgttgcgctcactgcccgctttccagtcgggaaacctgtcgtgccagctgcattaatgaatcggccaacgcgcggggagaggcggtttgcgtattgggcgctcttccgcttcctcgctcactgactcgctgcgctcggtcgttcggctgcggcgagcggtatcagctcactcaaaggcggtaatacggttatccacagaatcaggggataacgcaggaaagaacatgtgagcaaaaggccagcaaaaggccaggaaccgtaaaaaggccgcgttgctggcgtttttccataggctccgcccccctgacgagcatcacaaaaatcgacgctcaagtcagaggtggcgaaacccgacaggactataaagataccaggcgtttccccctggaagctccctcgtgcgctctcctgttccgaccctgccgcttaccggatacctgtccgcctttctcccttcgggaagcgtggcgctttctcaatgctcacgctgtaggtatctcagttcggtgtaggtcgttcgctccaagctgggctgtgtgcacgaaccccccgttcagcccgaccgctgcgccttatccggtaactatcgtcttgagtccaacccggtaagacacgacttatcgccactggcagcagccactggtaacaggattagcagagcgaggtatgtaggcggtgctacagagttcttgaagtggtggcctaactacggctacactagaaggacagtatttggtatctgcgctctgctgaagccagttaccttcggaaaaagagttggtagctcttgatccggcaaacaaaccaccgctggtagcggtggtttttttgtttgcaagcagcagattacgcgcagaaaaaaaggatctcaagaagatcctttgatcttttctacggggtctgacgctcagtggaacgaaaactcacgttaagggattttggtcatgagattatcaaaaaggatcttcacctagatccttttaaattaaaaatgaagttttaaatcaatctaaagtatatatgagtaaacttggtctgacagttaccaatgcttaatcagtgaggcacctatctcagcgatctgtctatttcgttcatccatagttgcctgactccccgtcgtgtagataactacgatacgggagggcttaccatctggccccagtgctgcaatgataccgcgagatccacgctcaccggctccagatttatcagcaataaaccagccagccggaagggccgagcgcagaagtggtcctgcaactttatccgcctccatccagtctattaattgttgccgggaagctagagtaagtagttcgccagttaatagtttgcgcaacgttgttgccattgctacaggcatcgtggtgtcacgctcgtcgtttggtatggcttcattcagctccggttcccaacgatcaaggcgagttacatgatcccccatgttgtgcaaaaaagcggttagctccttcggtcctccgatcgttgtcagaagtaagttggccgcagtgttatcactcatggttatggcagcactgcataattctcttactgtcatgccatccgtaagatgcttttctgtgactggtgagtactcaaccaagtcattctgagaatagtgtatgcggcgaccgagttgctcttgcccggcgtcaatacgggataataccgcgccacatagcagaactttaaaagtgctcatcattggaaaacgttcttcggggcgaaaactctcaaggatcttaccgctgttgagatccagttcgatgtaacccactcgtgcacccaactgatcttcagcatcttttactttcaccagcgtttctgggtgagcaaaaacaggaaggcaaaatgccgcaaaaaagggaataagggcgacacggaaatgttgaatactcatactcttcctttttcaatattattgaagcatttatcagggttattgtctcatgagcggatacatatttgaatgtatttagaaaaataaacaaataggggttccgcgcacatttccccgaaaagtgccacctgacgtcgacggatcgggagatctcccgatcccctatggtcgactctcagtacaatctgctctgatgccgcatagttaagccagtatctgctccctgcttgtgtgttggaggtcgctgagtagtgcgcgagcaaaatttaagctacaacaaggcaaggcttgaccgacaattgcatgaagaatctgcttagg

SEQ ID NO: 60 - DNA, 357 bp, synthetic construct
  source 1..357: mol_type = other DNA
caagtgcagctccagcagagcggcgccgagctggccagacctggagcttctgtgaaaatgagctgcaaggcctctggctataccttcaccagatacaccatgcactgggtcaagcagcggcctggccagggcctggaatggatcggctacatcaaccccagcagaggctacaccaattacaaccagaaattcaaggacaaggctacactgacaacagataagagcagctccaccgcctacatgcagctgagcagcctgaccagcgaggacagcgccgtgtactactgcgcccggtattacgacgaccactactgtctggattactggggccagggaacaaccctgaccgtgtcctct

SEQ ID NO: 61 - DNA, 366 bp, synthetic construct
  source 1..366: mol_type = other DNA
gaggtgcagctgcagcaaagcggacctgagctcgtgaagcctggagcctctatgaagatcagctgtaaagcctccggctacagctttaccggctatacaatgaactgggtcaagcagagccacggcaagaatctggaatggatgggcctgatcaacccctacaagggcgtgtccacctacaaccagaagttcaaggacaaggctacactgaccgtggacaaaagcagctctaccgcctacatggaactgctgagcctgacaagcgaggactccgccgtgtactactgcgccagaagcggctactacggcgattctgattggtacttcgacgtgtggggccagggcaccaccctgaccgtgttcagc

SEQ ID NO: 62 - DNA, 360 bp, synthetic construct
  source 1..360: mol_type = other DNA
gaggtgcaactggtggaaagcggcggaggactggtgcagcccggccggagcctgcggctgagctgtgccgcttctggttttaccttcagcaactacggcatggcctgggtcagacaggcccctggcaaaggcctcgagtgggtggctacaatcagctacgacggcagcatcacctactatagagatagcgtgaagggcagattcacaatctctagagataatagcaagaacaccctgtacctgcagatgaactctctgcgggccgaggacaccgccgtgtactactgcaccagagaggaacagtacagcagctggtacttcgacttctggggccagggcatcctggttacagtgtcctcc

SEQ ID NO: 63 - DNA, 363 bp, synthetic construct
  source 1..363: mol_type = other DNA
caagtgcagctgcagcagccaggagccgagctggtgaaacctggagctagcgtgaagatgagctgtaaagcctctggctacaccttcacctcttataatatgcactgggtcaagcagacccctggcagaggcctggaatggatcggcgctatctaccccggcaacggcgacaccagctacaaccagaagttcaagggcaaggccacactgacagccgacaagtccagctctacagcctacatgcagctgagcagcctgaccagcgaggacagcgccgtgtactactgcgcccggagcacctactacggcggagattggtactttaacgtgtggggcgccggcacaaccgtgaccgtgtccgcc

SEQ ID NO: 64 - DNA, 357 bp, synthetic construct
  source 1..357: mol_type = other DNA
caagtgcagctggtcgagagcggaggcggcgtggtgcagcctggaagaagcctgagactgagctgcgctgcttctggctttagcttcagctcttatgtgtgctgggtgcggcaggcccctggcaagggcctggaatggatcgcctgtatctacaccggcgacggcacaaattacagcgccagctgggccaagggcagattcaccatcagcaaggacagctctaaaaacacagtgtacctgcagatgaacagcctgcgggccgaggacaccgccgtgtacttctgcgccagaccagatatcacctacggcttcgccatcaacttctggggccccggaacactggtgaccgtgtcctcc

SEQ ID NO: 65 - DNA, 369 bp, synthetic construct
  source 1..369: mol_type = other DNA
caagtgcaactggtggaatctggaggaggactggtgcagcccggcggcagcctgaaactgagctgcgccgccagcggcttcgacttttctaggtactggatgagctgggtgcggcaggcccctggcaagggcctggaatggatcggcgagatcaatcctacaagcagcaccatcaacttcacccctagtctgaaggacaaggtgttcatcagccgcgacaacgccaagaacacactgtacctgcagatgagcaaggtgcggagcgaggacaccgccctctactactgcgccagaggcaactactacagatacggcgacgccatggactactggggccagggcacaagcgtgacagtgtccaaaatcagc

SEQ ID NO: 66 - DNA, 360 bp, synthetic construct
  source 1..360: mol_type = other DNA
caggtgcagctgaaacagagcggacctggcctggtccagcctagccagtccctgagcctgacatgcaccgtgtccggcttcagcctgaccagctacggcgtgcactgggtgcggcagcctcccggcaagggcctcgagtggctgggcgtgatctggtccggcggatctacagattacaacgccgcttttatcagcagactgagcatcagaaaggacaatagcaagagccaagtgttcttcaagatgaacagcctgcaggccgacgacaccgccatctactactgcgccagaaccttcaccacaagcaccagcgcctggttcgcctattggggccagggcaccctggtgaccgtgtctgct

SEQ ID NO: 67 - DNA, 321 bp, synthetic construct
  source 1..321: mol_type = other DNA
caaatcgtgctgacacagagccctgctatcatgagcgcctctccaggcgagaaggtcaccatgacctgtagcgccagcagcagcgtgtcctacatgaactggtaccagcagaaaagcggcaccagccccaagcggtggatctacgacaccagcaagctggcctccggcgtgcctgcccactttagaggcagcggatctggaacatcttatagcctgaccatcagcggcatggaagccgaggatgccgctacatactactgccagcagtggtcctctaatcctttcaccttcggcagcggcaccaagctggaaatcaacaga

SEQ ID NO: 68 - DNA, 324 bp, synthetic construct
  source 1..324: mol_type = other DNA
atggacattcagatgacccagaccaccagcagcctgagcgcttctctgggcgatagagtgaccatctcttgtagagccagccaggacatccggaactacctgaactggtatcagcagaaacctgatggcacagtgaagctgctgatctactacacctctagactgcacagcggcgtgcccagcaagttcagcggctccggcagcggaacagactacagcctcaccatctccaacctggagcaggaggacatcgccacatacttctgccagcaaggcaataccctgccttggacctttgccggcggaacaaagctggaaatcaag

SEQ ID NO: 69 - DNA, 333 bp, synthetic construct
  source 1..333: mol_type = other DNA
gatatccagctgacacagtctccatctagcctgagcgcctctgtgggcgatagagtgacaatcacctgtagagcctcccagagcgtgtccatcagcagccacgacctgatgcagtggtatcagcagaaacctggcaaggcccctaagctcctgatctacgacgccttcaacctggccagcggcgtccccagccggttcagcggatctggcagcggaaccgacttcaccctgaccattagctccctgcaacctgaggattttgctacatactactgccagcaaagcaaggacgacccctacaccttcggccagggcaccaagctggaaatcaag

SEQ ID NO: 70 - DNA, 318 bp, synthetic construct
  source 1..318: mol_type = other DNA
caaatcgtgctgtctcagagccctgctatcctgagcgcctctccaggcgagaaggtgaccatgacctgtagagccagctctagcgtgtcctatatccactggtttcagcagaaacctggcagcagccccaagccttggatctacgccaccagcaacctggccagcggcgtccccgtgcggttcagcggatctggctccggcaccagctacagcctgaccatcagcagagtggaagccgaggacgccgctacatactactgccagcagtggacctccaaccctcctacattcggcggcggaacaaagctggaaattaag

SEQ ID NO: 71 - DNA, 390 bp, synthetic construct
  source 1..390: mol_type = other DNA
atggacatgcgggtccccgcccagctgctcggcctgctgctgctgtggctgcgcggcgctagatgcgacatccagatgacccagtcccctagcagcctgagcgccagcgtgggcgatagagtgaccatcaagtgccaggccagccagagcatctcctccagactggcttggtatcagcagaagcccggcaagcctcctaagctgctgatctaccgggcctctacactggcctctggcgtgccatctagattcagcggcagcggatctggaacagatttcaccctgaccattagcagcctgcagcctgaggacgtggccacatactactgccaatgtaccggctacggcatcagctggcctatcggcggcggaaccaaggtggaaatcaaa

SEQ ID NO: 72 - DNA, 336 bp, synthetic construct
  source 1..336: mol_type = other DNA
agcgacatcgtgctgacccagagccctgcttctctggccgtgtctctgggccagcgggccacaattagctgtagagccagcaagtccgtgtccaccagcggttattcttacctgcactggtaccagcagaagcctggccagccacctaagctgctgatctacctggccagcaacctggaatctggcgtccccgctagattctctggaagcggcagtggcaccgatttcaccctgaacatccaccccgtggaggaagaagatgccgctacctactattgccagcacagcagagagctgccattcacatttggcagcggcaccaagctcgagatcaag

SEQ ID NO: 73 - DNA, 324 bp, synthetic construct
  source 1..324: mol_type = other DNA
tctatcgtgatgacccaaacacctaagttcctgctggtctccgccggagatagagtgaccatcacctgcaaggcttctcagagcgtgtccaacgacgtggcctggtatcagcaaaagcccggccagagccccaagctgctgatctactacgccagcaaccggtacaccggcgtgcctgatagattcacaggcagcggctacggcaccgacttcacatttaccatcagcaccgtgcaggccgaggacctggccgtgtacttctgccagcaggactacagcagccctccatggaccttcggcggaggcacaaagctggaaatcaga

SEQ ID NO: 74 - DNA, 990 bp, synthetic construct
  source 1..990: mol_type = other DNA
gccagcaccaagggtcccagcgtattccccctggccccaagtagcaaaagcaccagtggtggcacagcggccctcggatgcctggttaaggactatttccccgagccggtaaccgtaagctggaacagtggagcactgaccagcggcgtgcataccttccccgctgtactgcaatcctccggcctgtactcactgagcagcgtagtgacggtgccctctagcagcctgggcacccagacctacatctgcaacgtgaaccataaaccgtctaacacgaaggtcgacaaaaaagttgagcctaaaagctgcgacaagacccacacctgtcccccttgccccgctcccgagctgctgggaggcccctccgtgttcctgttccccccaaagcccaaagataccctgatgatcagcaggaccccggaggtgacctgcgtggtggtggacgtgagccacgaggaccctgaggtgaagttcaactggtacgtggacggcgtggaggttcacaacgccaagaccaaacccagggaggagcagtacaacagcacttacagggtggtgagcgtgctgaccgtgctgcaccaggactggctgaacggcaaggagtacaaatgcaaggttagcaacaaggcccttccagcccccatcgagaagaccatcagcaaggccaagggacagcctagggagccccaggtctacactctgccccccagccgcgacgagctgaccaagaaccaggtgagtttgacctgtctggtgaagggcttctaccccagcgacatcgccgtggagtgggagagcaacggccagcccgagaacaactacaaaaccaccccccctgtgctggactcagacggcagctttttcctgtattctaagctcaccgtggacaagagcaggtggcagcagggcaacgtgttcagttgcagcgtgatgcacgaggccctgcacaaccactacacccagaagagcttgagcctgagccccggaaag

SEQ ID NO: 75 - DNA, 321 bp, synthetic construct
  source 1..321: mol_type = other DNA
aggaccgtggctgcccccagcgtcttcatcttccccccgagcgacgagcagctgaagagcggcaccgccagcgtggtgtgcctgctgaacaacttctaccccagggaggccaaggtgcagtggaaggtggacaacgccctgcagagcggaaacagccaggagagcgtgaccgagcaggacagcaaggactctacttactccctgagcagcaccctgacactgagcaaggccgactacgagaagcacaaggtgtacgcctgcgaggtgacccaccagggcctgagctctcccgtgaccaagagcttcaacaggggcgagtgc

SEQ ID NO: 76 - DNA, 6141 bp, synthetic construct
  source 1..6141: mol_type = other DNA
gttaggcgttttgcgctgcttcgcgatgtacgggccagatatacgcgttgacattgattattgactagttattaatagtaatcaattacggggtcattagttcatagcccatatatggagttccgcgttacataacttacggtaaatggcccgcctggctgaccgcccaacgacccccgcccattgacgtcaataatgacgtatgttcccatagtaacgccaatagggactttccattgacgtcaatgggtggagtatttacggtaaactgcccacttggcagtacatcaagtgtatcatatgccaagtacgccccctattgacgtcaatgacggtaaatggcccgcctggcattatgcccagtacatgaccttatgggactttcctacttggcagtacatctacgtattagtcatcgctattaccatggtgatgcggttttggcagtacatcaatgggcgtggatagcggtttgactcacggggatttccaagtctccaccccattgacgtcaatgggagtttgttttggcaccaaaatcaacgggactttccaaaatgtcgtaacaactccgccccattgacgcaaatgggcggtaggcgtgtacggtgggaggtctatataagcagagctcgtttagtgaaccgtcagatcgcctggagacgccatccacgctgttttgacctccatagaagacaccgggaccgatccagcctccggactctagaggatcgaacccttgccaccatggaaaccgatacactgctgctgtgggtgctgttgctctgggttccaggctctaccggcggagaccttattagagctcatactccatatattaattttacaattgtgaacggtctcatgatgaaagggttcgatccctaccggttagtaatgagtttgatatctcgacaatcaacctctggattacaaaatttgtgaaagattgactggtattcttaactatgttgctccttttacgctatgtggatacgctgctttaatgcctttgtatcatgctattgcttcccgtatggctttcattttctcctccttgtataaatcctggttgctgtctctttatgaggagttgtggcccgttgtcaggcaacgtggcgtggtgtgcactgtgtttgctgacgcaacccccactggttggggcattgccaccacctgtcagctcctttccgggactttcgctttccccctccctattgccacggcggaactcatcgccgcctgccttgcccgctgctggacaggggctcggctgttgggcactgacaattccgtggtgttgtcggggaagctgacgtcctttccatggctgctcgcctgtgttgccacctggattctgcgcgggacgtccttctgctacgtcccttcggccctcaatccagcggaccttccttcccgcggcctgctgccggctctgcggcctcttccgcgtcttcgccttcgccctcagacgagtcggatctccctttgggccgcctccccgcctggaaacgggggaggctaactgaaacacggaaggagacaataccggaaggaacccgcgctatgacggcaataaaaagacagaataaaacgcacgggtgttgggtcgtttgttcataaacgcggggttcggtcccagggctggcactctgtcgataccccaccgtgaccccattggggccaatacgcccgcgtttcttccttttccccaccccaccccccaagttcgggtgaaggcccagggctcgcagccaacgtcggggcggcaggccctgccatagcagatctgcgcagctggggctctagggggtatccccacgcgccctgtagcggcgcattaagcgcggcgggtgtggtggttacgcgcagcgtgaccgctacacttgccagcgccctagcgcccgctcctttcgctttcttcccttcctttctcgccacgttcgccggctttccccgtcaagctctaaatcggggcatccctttagggttccgatttagtgctttacggcacctcgaccccaaaaaacttgattagggtgatggttcacgtagtgggccatcgccctgatagacggtttttcgccctttgacgttggagtccacgttctttaatagtggactcttgttccaaactggaacaacactcaaccctatctcggtctattcttttgatttataagggattttggggatttcggcctattggttaaaaaatgagctgatttaacaaaaatttaacgcgaattaattctgtggaatgtgtgtcagttagggtgtggaaagtccccaggctccccagcaggcagaagtatgcaaagcatgcatctcaattagtcagcaaccaggtgtggaaagtccccaggctccccagcaggcagaagtatgcaaagcatgcatctcaattagtcagcaaccatagtcccgcccctaactccgcccatcccgcccctaactccgcccagttccgcccattctccgccccatggctgactaattttttttatttatgcagaggccgaggccgcctctgcctctgagctattccagaagtagtgaggaggcttttttggaggcctaggcttttgcaaaaagctcccgggagcttgtatatccattttcggatctgatcaagagacaggatgaggatcgtttcgcatgattgaacaagatggattgcacgcaggttctccggccgcttgggtggagaggctattcggctatgactgggcacaacagacaatcggctgctctgatgccgccgtgttccggctgtcagcgcaggggcgcccggttctttttgtcaagaccgacctgtccggtgccctgaatgaactgcaggacgaggcagcgcggctatcgtggctggccacgacgggcgttccttgcgcagctgtgctcgacgttgtcactgaagcgggaagggactggctgctattgggcgaagtgccggggcaggatctcctgtcatctcaccttgctcctgccgagaaagtatccatcatggctgatgcaatgcggcggctgcatacgcttgatccggctacctgcccattcgaccaccaagcgaaacatcgcatcgagcgagcacgtactcggatggaagccggtcttgtcgatcaggatgatctggacgaagagcatcaggggctcgcgccagccgaactgttcgccaggctcaaggcgcgcatgcccgacggcgaggatctcgtcgtgacccatggcgatgcctgcttgccgaatatcatggtggaaaatggccgcttttctggattcatcgactgtggccggctgggtgtggcggaccgctatcaggacatagcgttggctacccgtgatattgctgaagagcttggcggcgaatgggctgaccgcttcctcgtgctttacggtatcgccgctcccgattcgcagcgcatcgccttctatcgccttcttgacgagttcttctgagcgggactctggggttcgcgaaatgaccgaccaagcgacgcccaacctgccatcacgagatttcgattccaccgccgccttctatgaaaggttgggcttcggaatcgttttccgggacgccggctggatgatcctccagcgcggggatctcatgctggagttcttcgcccaccccaacttgtttattgcagcttataatggttacaaataaagcaatagcatcacaaatttcacaaataaagcatttttttcactgcattctagttgtggtttgtccaaactcatcaatgtatcttatcatgtctgtataccgtcgacctctagctagagcttggcgtaatcatggtcatagctgtttcctgtgtgaaattgttatccgctcacaattccacacaacatacgagccggaagcataaagtgtaaagcctggggtgcctaatgagtgagctaactcacattaattgcgttgcgctcactgcccgctttccagtcgggaaacctgtcgtgccagctgcattaatgaatcggccaacgcgcggggagaggcggtttgcgtattgggcgctcttccgcttcctcgctcactgactcgctgcgctcggtcgttcggctgcggcgagcggtatcagctcactcaaaggcggtaatacggttatccacagaatcaggggataacgcaggaaagaacatgtgagcaaaaggccagcaaaaggccaggaaccgtaaaaaggccgcgttgctggcgtttttccataggctccgcccccctgacgagcatcacaaaaatcgacgctcaagtcagaggtggcgaaacccgacaggactataaagataccaggcgtttccccctggaagctccctcgtgcgctctcctgttccgaccctgccgcttaccggatacctgtccgcctttctcccttcgggaagcgtggcgctttctcaatgctcacgctgtaggtatctcagttcggtgtaggtcgttcgctccaagctgggctgtgtgcacgaaccccccgttcagcccgaccgctgcgccttatccggtaactatcgtcttgagtccaacccggtaagacacgacttatcgccactggcagcagccactggtaacaggattagcagagcgaggtatgtaggcggtgctacagagttcttgaagtggtggcctaactacggctacactagaaggacagtatttggtatctgcgctctgctgaagccagttaccttcggaaaaagagttggtagctcttgatccggcaaacaaaccaccgctggtagcggtggtttttttgtttgcaagcagcagattacgcgcagaaaaaaaggatctcaagaagatcctttgatcttttctacggggtctgacgctcagtggaacgaaaactcacgttaagggattttggtcatgagattatcaaaaaggatcttcacctagatccttttaaattaaaaatgaagttttaaatcaatctaaagtatatatgagtaaacttggtctgacagttaccaatgcttaatcagtgaggcacctatctcagcgatctgtctatttcgttcatccatagttgcctgactccccgtcgtgtagataactacgatacgggagggcttaccatctggccccagtgctgcaatgataccgcgagatccacgctcaccggctccagatttatcagcaataaaccagccagccggaagggccgagcgcagaagtggtcctgcaactttatccgcctccatccagtctattaattgttgccgggaagctagagtaagtagttcgccagttaatagtttgcgcaacgttgttgccattgctacaggcatcgtggtgtcacgctcgtcgtttggtatggcttcattcagctccggttcccaacgatcaaggcgagttacatgatcccccatgttgtgcaaaaaagcggttagctccttcggtcctccgatcgttgtcagaagtaagttggccgcagtgttatcactcatggttatggcagcactgcataattctcttactgtcatgccatccgtaagatgcttttctgtgactggtgagtactcaaccaagtcattctgagaatagtgtatgcggcgaccgagttgctcttgcccggcgtcaatacgggataataccgcgccacatagcagaactttaaaagtgctcatcattggaaaacgttcttcggggcgaaaactctcaaggatcttaccgctgttgagatccagttcgatgtaacccactcgtgcacccaactgatcttcagcatcttttactttcaccagcgtttctgggtgagcaaaaacaggaaggcaaaatgccgcaaaaaagggaataagggcgacacggaaatgttgaatactcatactcttcctttttcaatattattgaagcatttatcagggttattgtctcatgagcggatacatatttgaatgtatttagaaaaataaacaaataggggttccgcgcacatttccccgaaaagtgccacctgacgtcgacggatcgggagatctcccgatcccctatggtcgactctcagtacaatctgctctgatgccgcatagttaagccagtatctgctccctgcttgtgtgttggaggtcgctgagtagtgcgcgagcaaaatttaagctacaacaaggcaaggcttgaccgacaattgcatgaagaatctgcttagg

SEQ ID NO: 77 - DNA, 35 bp, synthetic construct
  source 1..35: mol_type = other DNA
accggtgtacattctgtgacctgcaagtccggcga

SEQ ID NO: 78 - DNA, 34 bp, synthetic construct
  source 1..34: mol_type = other DNA
cggatccaccacctcccacaggacagctggcctc

SEQ ID NO: 79 - DNA, 38 bp, synthetic construct
  source 1..38: mol_type = other DNA
ggaggtggtggatccgagcccaaatcttgtgacaaaac

SEQ ID NO: 80 - DNA, 29 bp, synthetic construct
  source 1..29: mol_type = other DNA
tccagagcctttacccggggacagggaga

SEQ ID NO: 81 - DNA, 38 bp, synthetic construct
  source 1..38: mol_type = other DNA
ggtaaaggctctggaggtgatcagaatcctcaaattgc

SEQ ID NO: 82 - DNA, 35 bp, synthetic construct
  source 1..35: mol_type = other DNA
cggccgtcgcactcagagtttgagtaagccaaagg

SEQ ID NO: 83 - DNA, 9180 bp, synthetic construct
  source 1..9180: mol_type = other DNA
gacggatcgggagatctcccgatcccctatggtcgactctcagtacaatctgctctgatgccgcatagttaagccagtatctgctccctgcttgtgtgttggaggtcgctgagtagtgcgcgagcaaaatttaagctacaacaaggcaaggcttgaccgacaattgcatgaagaatctgcttagggttaggcgttttgcgctgcttcgcgatgtacgggccagatatacgcgttgacattgattattgactagttattaatagtaatcaattacggggtcattagttcatagcccatatatggagttccgcgttacataacttacggtaaatggcccgcctggctgaccgcccaacgacccccgcccattgacgtcaataatgacgtatgttcccatagtaacgccaatagggactttccattgacgtcaatgggtggactatttacggtaaactgcccacttggcagtacatcaagtgtatcatatgccaagtacgccccctattgacgtcaatgacggtaaatggcccgcctggcattatgcccagtacatgaccttatgggactttcctacttggcagtacatctacgtattagtcatcgctattaccatggtgatgcggttttggcagtacatcaatgggcgtggatagcggtttgactcacggggatttccaagtctccaccccattgacgtcaatgggagtttgttttggcaccaaaatcaacgggactttccaaaatgtcgtaacaactccgccccattgacgcaaatgggcggtaggcgtgtacggtgggaggtctatataagcagcgcgttttgcctgtactgggtctctctggttagaccagatctgagcctgggagctctctggctaactagggaacccactgcttaagcctcaataaagcttgccttgagtgcttcaagtagtgtgtgcccgtctgttgtgtgactctggtaactagagatccctcagacccttttagtcagtgtggaaaatctctagcagtggcgcccgaacagggacctgaaagcgaaagggaaaccagagctctctcgacgcaggactcggcttgctgaagcgcgcacggcaagaggcgaggggcggcgactggtgagtacgccaaaaattttgactagcggaggctagaaggagagagatgggtgcgagagcgtcagtattaagcgggggagaattagatcgcgatgggaaaaaattcggttaaggccagggggaaagaaaaaatataaattaaaacatatagtatgggcaagcagggagctagaacgattcgcagttaatcctggcctgttagaaacatcagaaggctgtagacaaatactgggacagctacaaccatcccttcagacaggatcagaagaacttagatcattatataatacagtagcaaccctctattgtgtgcatcaaaggatagagataaaagacaccaaggaagctttagacaagatagaggaagagcaaaacaaaagtaagaccaccgcacagcaagcggccgctgatcttcagacttggaggaggagatatgagggacaattggagaagtgaattatataaatataaagtagtaaaaattgaaccattaggagtagcacccaccaaggcaaagagaagagtggtgcagagagaaaaaagagcagtgggaataggagctttgttccttgggttcttgggagcagcaggaagcactatgggcgcagcctcaatgacgctgacggtacaggccagacaattattgtctggtatagtgcagcagcagaacaatttgctgagggctattgaggcgcaacagcatctgttgcaactcacagtctggggcatcaagcagctccaagcaagaatcctagctgtggaaagatacctaaaggatcaacagctcctagggatttggggttgctctggaaaactcatttgcaccactgctgtgccttggaatgctagttggagtaataaatctctggaacagatctggaatcacacgacctggatggagtgggacagagaaattaacaattacacaagcttaatacactccttaattgaagaatcgcaaaaccagcaagaaaagaatgaacaagaattattggaattagataaatgggcaagtttgtggaattggtttaacataacaaattggctgtggtatataaaattattcataatgatagtaggaggcttggtaggtttaagaatagtttttgctgtactttctatagtgaatagagttaggcagggatattcaccattatcgtttcagacccacctcccaatcccgaggggacccgacaggcccgaaggaatagaagaagaaggtggagagagagacagagacagatccattcgattagtgaacggatcaacttttaaaagaaaaggggggattggggggtacagtgcaggggaaagaatagtagacataatagcaacagacatacaaactaaagaattacaaaaacaaattacaaaaattcaaaattttatcgataagcttgggagttccgcgttacataacttacggtaaatggcccgcctggctgaccgcccaacgacccccgcccattgacgtcaataatgacgtatgttcccatagtaacgccaatagggactttccattgacgtcaatgggtggagtatttacggtaaactgcccacttggcagtacatcaagtgtatcatatgccaagtacgccccctattgacgtcaatgacggtaaatggcccgcctggcattatgcccagtacatgaccttatgggactttcctacttggcagtacatctacgtattagtcatcgctattaccatggtgatgcggttttggcagtacatcaatgggcgtggatagcggtttgactcacggggatttccaagtctccaccccattgacgtcaatgggagtttgttttggcaccaaaatcaacgggactttccaaaatgtcgtaacaactccgccccattgacgcaaatgggcggtaggcgtgtacggtgggaggtctatataagcagagctcgtttagtgaaccgtcagatcgcctggagacgccatccacgctgttttgacctccatagaagacaccgactctagaggatccaccggtcgccaccatggtgagcaagggcgaggagctgttcaccggggtggtgcccatcctggtcgagctggacggcgacgtaaacggccacaagttcagcgtgtccggcgagggcgagggcgatgccacctacggcaagctgaccctgaagttcatctgcaccaccggcaagctgcccgtgccctggcccaccctcgtgaccaccctgacctacggcgtgcagtgcttcagccgctaccccgaccacatgaagcagcacgacttcttcaagtccgccatgcccgaaggctacgtccaggagcgcaccatcttcttcaaggacgacggcaactacaagacccgcgccgaggtgaagttcgagggcgacaccctggtgaaccgcatcgagctgaagggcatcgacttcaaggaggacggcaacatcctggggcacaagctggagtacaactacaacagccacaacgtctatatcatggccgacaagcagaagaacggcatcaaggtgaacttcaagatccgccacaacatcgaggacggcagcgtgcagctcgccgaccactaccagcagaacacccccatcggcgacggccccgtgctgctgcccgacaaccactacctgagcacccagtccgccctgagcaaagaccccaacgagaagcgcgatcacatggtcctgctggagttcgtgaccgccgccgggatcactctcggcatggacgagctgtacaagtaaagcggccgcgtcgagtttaaacctggaaaaacatggagcaatcacaagtagcaacacagcagctaccaatgctgcttgtgcctggctagaagcacaagaggaggaggaggtgggttttccagtcacacctcagacaatcaacctctggattacaaaatttgtgaaagattgactggtattcttaactatgttgctccttttacgctatgtggatacgctgctttaatgcctttgtatcatgctattgcttcccgtatggctttcattttctcctccttgtataaatcctggttgctgtctctttatgaggagttgtggcccgttgtcaggcaacgtggcgtggtgtgcactgtgtttgctgacgcaacccccactggttggggcattgccaccacctgtcagctcctttccgggactttcgctttccccctccctattgccacggcggaactcatcgccgcctgccttgcccgctgctggacaggggctcggctgttgggcactgacaattccgtggtgttgtcggggaagctgacgtcctttccatggctgctcgcctgtgttgccacctggattctgcgcgggacgtccttctgctacgtcccttcggccctcaatccagcggaccttccttcccgcggcctgctgccggctctgcggcctcttccgcgtcttcgccttcgccctcagacgagtcggatctccctttgggccgcctccccgcctggaattcgagctcggtacctttaagaccaatgacttacaaggcagctgtagatcttagccactttttaaaagaaaaggggggactggaagggctaattcactcccaaagaagacaagatatccttgatctgtggatctaccacacacaaggctacttccctgattgacagaactacacaccagggccaggggtcagatatccactgacctttggatggtgctacaagctagtaccagttgagccagataagatagaagaggccaataaaggagagaacaccagcttgttacaccctgtgagcctgcatgggatggatgacccggagagagaagtgttagagtggaggtttgacagccgcctagcatttcatcacgtggcccgagagctgcatccggactgtactgggtctctctggttagaccagatctgagcctgggagctctctggctaactagggaacccactgcttaagcctcaataaagcttgccttgagtgcttcaagtagtgtgtgcccgtctgttgtgtgactctggtaactagagatccctcagacccttttagtcagtgtggaaaatctctagcagggccgctttaaacccgctgatcagcctcgactgtgccttctagttgccagccatctgttgtttgcccctcccccgtgccttccttgaccctggaaggtgccactcccactgtcctttcctaataaaatgaggaaattgcatcgcattgtctgagtaggtgtcattctattctggggggtggggtggggcaggacagcaagggggaggattgggaagacaatagcaggcatgctggggatgcggtgggctctatggcttctgaggcggaaagaaccagctggggctctagggggtatccccacgcgccctgtagcggcgcattaagcgcggcgggtgtggtggttacgcgcagcgtgaccgctacacttgccagcgccctagcgcccgctcctttcgctttcttcccttcctttctcgccacgttcgccggctttccccgtcaagctctaaatcggggcatccctttagggttccgatttagtgctttacggcacctcgaccccaaaaaacttgattagggtgatggttcacgtagtgggccatcgccctgatagacggtttttcgccctttgacgttggagtccacgttctttaatagtggactcttgttccaaactggaacaacactcaaccctatctcggtctattcttttgatttataagggattttggggatttcggcctattggttaaaaaatgagctgatttaacaaaaatttaacgcgaattaattctgtggaatgtgtgtcagttagggtgtggaaagtccccaggctccccaggcaggcagaagtatgcaaagcatgcatctcaattagtcagcaaccaggtgtggaaagtccccaggctccccagcaggcagaagtatgcaaagcatgcatctcaattagtcagcaaccatagtcccgcccctaactccgcccatcccgcccctaactccgcccagttccgcccattctccgccccatggctgactaattttttttatttatgcagaggccgaggccgcctctgcctctgagctattccagaagtagtgaggaggcttttttggaggcctaggcttttgcaaaaagctcccgggagcttgtatatccattttcggatctgatcagcacgtgttgacaattaatcatcggcatagtatatcggcatagtataatacgacaaggtgaggaactaaaccatggccaagttgaccagtgccgttccggtgctcaccgcgcgcgacgtcgccggagcggtcgagttctggaccgaccggctcgggttctcccgggacttcgtggaggacgacttcgccggtgtggtccgggacgacgtgaccctgttcatcagcgcggtccaggaccaggtggtgccggacaacaccctggcctgggtgtgggtgcgcggcctggacgagctgtacgccgagtggtcggaggtcgtgtccacgaacttccgggacgcctccgggccggccatgaccgagatcggcgagcagccgtgggggcgggagttcgccctgcgcgacccggccggcaactgcgtgcacttcgtggccgaggagcaggactgacacgtgctacgagatttcgattccaccgccgccttctatgaaaggttgggcttcggaatcgttttccgggacgccggctggatgatcctccagcgcggggatctcatgctggagttcttcgcccaccccaacttgtttattgcagcttataatggttacaaataaagcaatagcatcacaaatttcacaaataaagcatttttttcactgcattctagttgtggtttgtccaaactcatcaatgtatcttatcatgtctgtataccgtcgacctctagctagagcttggcgtaatcatggtcatagctgtttcctgtgtgaaattgttatccgctcacaattccacacaacatacgagccggaagcataaagtgtaaagcctggggtgcctaatgagtgagctaactcacattaattgcgttgcgctcactgcccgctttccagtcgggaaacctgtcgtgccagctgcattaatgaatcggccaacgcgcggggagaggcggtttgcgtattgggcgctcttccgcttcctcgctcactgactcgctgcgctcggtcgttcggctgcggcgagcggtatcagctcactcaaaggcggtaatacggttatccacagaatcaggggataacgcaggaaagaacatgtgagcaaaaggccagcaaaaggccaggaaccgtaaaaaggccgcgttgctggcgtttttccataggctccgcccccctgacgagcatcacaaaaatcgacgctcaagtcagaggtggcgaaacccgacaggactataaagataccaggcgtttccccctggaagctccctcgtgcgctctcctgttccgaccctgccgcttaccggatacctgtccgcctttctcccttcgggaagcgtggcgctttctcaatgctcacgctgtaggtatctcagttcggtgtaggtcgttcgctccaagctgggctgtgtgcacgaaccccccgttcagcccgaccgctgcgccttatccggtaactatcgtcttgagtccaacccggtaagacacgacttatcgccactggcagcagccactggtaacaggattagcagagcgaggtatgtaggcggtgctacagagttcttgaagtggtggcctaactacggctacactagaaggacagtatttggtatctgcgctctgctgaagccagttaccttcggaaaaagagttggtagctcttgatccggcaaacaaaccaccgctggtagcggtggtttttttgtttgcaagcagcagattacgcgcagaaaaaaaggatctcaagaagatcctttgatcttttctacggggtctgacgctcagtggaacgaaaactcacgttaagggattttggtcatgagattatcaaaaaggatcttcacctagatccttttaaattaaaaatgaagttttaaatcaatctaaagtatatatgagtaaacttggtctgacagttaccaatgcttaatcagtgaggcacctatctcagcgatctgtctatttcgttcatccatagttgcctgactccccgtcgtgtagataactacgatacgggagggcttaccatctggccccagtgctgcaatgataccgcgagacccacgctcaccggctccagatttatcagcaataaaccagccagccggaagggccgagcgcagaagtggtcctgcaactttatccgcctccatccagtctattaattgttgccgggaagctagagtaagtagttcgccagttaatagtttgcgcaacgttgttgccattgctacaggcatcgtggtgtcacgctcgtcgtttggtatggcttcattcagctccggttcccaacgatcaaggcgagttacatgatcccccatgttgtgcaaaaaagcggttagctccttcggtcctccgatcgttgtcagaagtaagttggccgcagtgttatcactcatggttatggcagcactgcataattctcttactgtcatgccatccgtaagatgcttttctgtgactggtgagtactcaaccaagtcattctgagaatagtgtatgcggcgaccgagttgctcttgcccggcgtcaatacgggataataccgcgccacatagcagaactttaaaagtgctcatcattggaaaacgttcttcggggcgaaaactctcaaggatcttaccgctgttgagatccagttcgatgtaacccactcgtgcacccaactgatcttcagcatcttttactttcaccagcgtttctgggtgagcaaaaacaggaaggcaaaatgccgcaaaaaagggaataagggcgacacggaaatgttgaatactcatactcttcctttttcaatattattgaagcatttatcagggttattgtctcatgagcggatacatatttgaatgtatttagaaaaataaacaaataggggttccgcgcacatttccccgaaaagtgccacctgacgtc

SEQ ID NO: 84 - DNA, 5822 bp, synthetic construct
  source 1..5822: mol_type = other DNA
attaggcagaatccagatgctcaaggcccttcataatatcccccagtttagtagttggacttagggaacaaaggaacctttaatagaaattggacagcaagaaagcgagcttagtgatacttgtgggccagggcattagccacaccagccaccactttctgataggcagcctgcactggtggggtgaattccgtttttttttttttttttcataaaaattaaaaactcaaatataattgaggcctctttgagcatggtatcacaagttgatttggtccaaacatgaagaatctgttgtgcaggatttgagttactttccaagtcggttcatctctatgtctgtataaatctgtcttttcttggtgtgctttaatttaatgcaaagatggataccaactcggagaaccaagaatagtccaatgattaaccctatgataaagaaaaaagaggcaatagagcttttccaactactgaaccaaccttctacaagctcgattggatttttggatagcccagtatcaccaaaaaataaactctcatcatcaggaagttgcgaagcagcgtcttgaatgtgaggatgttcgaacacctgagcctttgagctaagatgaagatcggagtccaacataccatgtccaatcatgtataaaggaaacttatatcctgaactggtcctcagaactccattgggtccaatttccacgtcttcatatggtgcccagtcatcccacagttccctttctgtggtagttccactgatcattccgaccattcttgagaggattggagcagcaatatcgactctgatgtatctggtctcaaagtattttagggtaccattgattatggtgaaagcaggaccggttcctgggtttttaggagcaagatagctgagatccactggagagattggaagacccgctctgattttgctccaggtttcttggcagagggaataatccaagatcctctcaacgtcctgaattagacttacatccactgaggtctgagatggagcagagatacttgacccttctgggcattcagggaatctggctgcagcaaagagatccttatcagccatctcgaaccagacacctgatgggagtctgactccccaatgcttgcagtattgcattttgcaggccttgcctccagtttcataagcaaagtagttacttctgaaccctgtgccctcctttcccagggatgatagctctccgtcctctgagaagaaggtgatgtccatggaaatgaggttagaatcacatagccctttgaccttatagtcagaatgccaggttgtagagttatggacagtggggcatatgtaattgctgcattttccgttgatgaactgtgaatcaacccattctcctgtgtattcatcaaccagcacatggtgaggagtcacctggacaatcactgcttcggcatccgtcacagttgcatatccacaactttgaggagggaagcctggattcagccaagttccttgtttcgtttgttcaatgctttccttgcattgttctacagatggagtgaaggatcggatggaatgtgttatatacttcggtccataccagcggaaatcacaagtagtgacccatttggaagcatgacacatccaaccgtctgcttgaatagccttgtgactcttgggcattttgacttgtaaggctgtgcctattaagtcattatgccaatttaaatctgagcttgacgggcaataatggtaattagaaggaacatttttccagtttcctttttggttgtgtggaaaaactatggtgaacttgcaattcaccccaatgaataaaaaggctaagtacaaaaggcacttcatagtgtcagaattcagatctcacgtgctttgccaaagtgatgggccagcacacagaccagcacgttgcccaggagctgtgggaggaagataagaggtatgaacatgattagcaaaagggcctagcttggactcagaataatccagccttatcccaaccataaaataaaagcagaatggtagctggattgtagctgctattagcaatatgaaacctcttacatcagttacaatttatatgcagaaatatttatatgcagaaatattgctattgccttaacccagaaattatcactgttattctttagaatggtgcaaagaggcatgatacattgtatcattattgccctgaaagaaagagattagggaaagtattagaaataagataaacaaaaaagtatattaaaagaagaaagcattttttaaaattacaaatgcaaaattaccctgatttggtcaatatgtgtaccctgttacttctccccttcctatgacatgaacttaaccatagaaaagaaggggaaagaaaacatcaagggtcccatagactcaccctgaagttctcaggatccgagctcggtaccacatgtaagcttcgaggggaggctggatcggtcccggtgtcttctatggaggtcaaaacagcgtggatggcgtctccaggcgatctgacggttcactaaacgagctctgcttatatagacctcccaccgtacacgcctaccgcccatttgcgtcaatggggcggagttgttacgacattttggaaagtcccgttgattttggtgccaaaacaaactcccattgacgtcaatggggtggagacttggaaatccccgtgagtcaaaccgctatccacgcccattgatgtactgccaaaaccgcatcaccatggtaatagcgatgactaatacgtagatgtactgccaagtaggaaagtcccataaggtcatgtactgggcataatgccaggcgggccatttaccgtcattgacgtcaatagggggcgtacttggcatatgatacacttgatgtactgccaagtgggcagtttaccgtaaatactccacccattgacgtcaatggaaagtccctattggcgttactatgggaacatacgtcattattgacgtcaatgggcgggggtcgttgggcggtcagccaggcgggccatttaccgtaagttatgtaacgcggaactccatatatgggctatgaactaatgaccccgtaattgattactattaataactagtcaataatcaatgtcaacatggcggtaatgttggacatgagccaatataaatgtacatattatgatatggatacaacgtatgcaatgggccaagctcatggctgactaattttttttatttatgcagaggccgaggccggatcctctagcccatgggggccccctcaggggatccacgtcaggtggcacttttcggggaaatgtgcgcggaacccctatttgtttatttttctaaatacattcaaatatgtatccgctcatgagacaataaccctgataaatgcttcaataatattgaaaaaggaagagtatgagtattcaacatttccgtgtcgcccttattcccttttttgcggcattttgccttcctgtttttgctcacccagaaacgctggtgaaagtaaaagatgctgaagatcagttgggtgcacgagtgggttacatcgaactggatctcaacagcggtaagatccttgagagttttcgccccgaagaacgttttccaatgatgagcacttttaaagttctgctatgtggcgcggtattatcccgtattgacgccgggcaagagcaactcggtcgccgcatacactattctcagaatgacttggttgagtactcaccagtcacagaaaagcatcttacggatggcatgacagtaagagaattatgcagtgctgccataaccatgagtgataacactgcggccaacttacttctgacaacgatcggaggaccgaaggagctaaccgcttttttgcacaacatgggggatcatgtaactcgccttgatcgttgggaaccggagctgaatgaagccataccaaacgacgagcgtgacaccacgatgcctgtagcaatggcaacaacgttgcgcaaactattaactggcgaactacttactctagcttcccggcaacaattaatagactggatggaggcggataaagttgcaggaccacttctgcgctcggcccttccggctggctggtttattgctgataaatctggagccggtgagcgtgggtctcgcggtatcattgcagcactggggccagatggtaagccctcccgtatcgtagttatctacacgacggggagtcaggcaactatggatgaacgaaatagacagatcgctgagataggtgcctcactgattaagcattggtaactgtcagaccaagtttactcatatatactttagattgatttaaaacttcatttttaatttaaaaggatctaggtgaagatcctttttgataatctcatgaccaaaatcccttaacgtgagttttcgttccactgagcgtcagaccccgtagaaaagatcaaaggatcttcttgagatcctttttttctgcgcgtaatctgctgcttgcaaacaaaaaaaccaccgctaccagcggtggtttgtttgccggatcaagagctaccaactctttttccgaaggtaactggcttcagcagagcgcagataccaaatactgttcttctagtgtagccgtagttaggccaccacttcaagaactctgtagcaccgcctacatacctcgctctgctaatcctgttaccagtggctgctgccagtggcgataagtcgtgtcttaccgggttggactcaagacgatagttaccggataaggcgcagcggtcgggctgaacggggggttcgtgcacacagcccagcttggagcgaacgacctacaccgaactgagatacctacagcgtgagctatgagaaagcgccacgcttcccgaagggagaaaggcggacaggtatccggtaagcggcagggtcggaacaggagagcgcacgagggagcttccagggggaaacgcctggtatctttatagtcctgtcgggtttcgccacctctgacttgagcgtcgatttttgtgatgctcgtcaggggggcggagcctatggaaaaacgccagcaacgcggcctttttacggttcctggccttttgctggccttttgctcacatgttctttcctgcgttatcccctgattctgtggataaccgtattaccgcctttgagtgagctgataccgctcgccgcagccgaacgaccgagcgcagcgagtcagtgagcgaggaagcagatctgcggccgcactagtgctagactgccatgtcgagggattccgggtcactgtgagtgggggaggcagggaagaagggctcacaggacagtcaaaccatgccccctgtttttccttcttcaagtagacctctataagacaacagagacaactaaggctgagtggccaggcgaggagaaaccatctcgccgtaaaacatggaaggaacacttcaggggaaaggtggtatctctaagcaagagaactgagtggagtcaaggctgagagatgcaggataagcaaatgggtagtgaaaagacattcatgaggacagctaaaacaataagtaatgtaaaatacagcatagcaaaactttaacctccaaatcaagcctctacttgaatccttttctgagggatgaataaggcataggcatcaggggctgttgccaatgtgcattagctgtttgcagcctcaccttctttcatggagtttaagatatagtgtattttcccaaggtttgaactagctcttcatttctttatgttttaaatgcactgacctcccacattccctttttagtaaaatattcagaaataatttaaatacatcattgcaatgaaaataaatgtttttt

SEQ ID NO: 85 - DNA, 4180 bp, synthetic construct
  source 1..4180: mol_type = other DNA
agcttggagcgaacgacctacaccgaactgagatacctacagcgtgagctatgagaaagcgccacgcttcccgaagggagaaaggcggacaggtatccggtaagcggcagggtcggaacaggagagcgcacgagggagcttccagggggaaacgcctggtatctttatagtcctgtcgggtttcgccacctctgacttgagcgtcgatttttgtgatgctcgtcaggggggcggagcctatggaaaaacgccagcaacgcggcctttttacggttcctggccttttgctggccttttgctcacatgttctttcctgcgttatcccctgattctgtggataaccgtattaccgcctttgagtgagctgataccgctcgccgcagccgaacgaccgagcgcagcgagtcagtgagcgaggaagcggaagagcgcccaatacgcaaaccgcctctccccgcgcgttggccgattcattaatgcagctggcacgacaggtttcccgactggaaagcgggcagtgagcgcaacgcaattaatgtgagttagctcactcattaggcaccccaggctttacactttatgcttccggctcgtatgttgtgtggaattgtgagcggataacaatttcacacaggaaacagctatgacatgattacgaattcgatgtacgggccagatatacgcgtatctgaggggactagggtgtgtttaggcgaaaagcggggcttcggttgtacgcggttaggagtcccctcaggatatagtagtttcgcttttgcatagggagggggaaatgtagtcttatgcaatactcttgtagtcttgcaacatggtaacgatgagttagcaacatgccttacaaggagagaaaaagcaccgtgcatgccgattggtggaagtaaggtggtacgatcgtgccttattaggaaggcaacagacgggtctgacatggattggacgaaccactgaattccgcattgcagagatattgtatttaagtgcctagctcgatacaataaacgccatttgaccattcaccacattggtgtgcacctccaagctcgagctcgtttagtgaaccgtcagatcgcctggagacgccatccacgctgttttgacctccatagaagacaccgggaccgatccagcctcccctcgaagctagtcgattaggcatctcctatggcaggaagaagcggagacagcgacgaagacctcctcaaggcagtcagactcatcaagtttctctatcaaagcaacccacctcccaatcccgaggggacccgacaggcccgaaggaatagaagaagaaggtggagagagagacagagacagatccattcgattagtgaacggatccttagcacttatctgggacgatctgcggagcctgtgcctcttcagctaccaccgcttgagagacttactcttgattgtaacgaggattgtggaacttctgggacgcagggggtgggaagccctcaaatattggtggaatctcctacaatattggagtcaggagctaaagaatagtgctgttagcttgctcaatgccacagctatagcagtagctgaggggacagatagggttatagaagtagtacaagaagcttggcactggccgtcgttttacaacgtcgtgatctgagcctgggagatctctggctaactagggaacccactgcttaagcctcaataaagcttgccttgagtgcttcaagtagtgtgtgcccgtctgttgtgtgactctggtaactagagatcaggaaaaccctggcgttacccaacttaatcgccttgcagcacatccccctttcgccagctggcgtaatagcgaagaggcccgcaccgatcgcccttcccaacagttgcgcagcctgaatggcgaatggcgcctgatgcggtattttctccttacgcatctgtgcggtatttcacaccgcatacgtcaaagcaaccatagtacgcgccctgtagcggcgcattaagcgcggcgggtgtggtggttacgcgcagcgtgaccgctacacttgccagcgccctagcgcccgctcctttcgctttcttcccttcctttctcgccacgttcgccggctttccccgtcaagctctaaatcgggggctccctttagggttccgatttagtgctttacggcacctcgaccccaaaaaacttgatttgggtgatggttcacgtagtgggccatcgccctgatagacggtttttcgccctttgacgttggagtccacgttctttaatagtggactcttgttccaaactggaacaacactcaaccctatctcgggctattcttttgatttataagggattttgccgatttcggcctattggttaaaaaatgagctgatttaacaaaaatttaacgcgaattttaacaaaatattaacgtttacaattttatggtgcactctcagtacaatctgctctgatgccgcatagttaagccagccccgacacccgccaacacccgctgacgcgccctgacgggcttgtctgctcccggcatccgcttacagacaagctgtgaccgtctccgggagctgcatgtgtcagaggttttcaccgtcatcaccgaaacgcgcgagacgaaagggcctcgtgatacgcctatttttataggttaatgtcatgataataatggtttcttagacgtcaggtggcacttttcggggaaatgtgcgcggaacccctatttgtttatttttctaaatacattcaaatatgtatccgctcatgagacaataaccctgataaatgcttcaataatattgaaaaaggaagagtatgagtattcaacatttccgtgtcgcccttattcccttttttgcggcattttgccttcctgtttttgctcacccagaaacgctggtgaaagtaaaagatgctgaagatcagttgggtgcacgagtgggttacatcgaactggatctcaacagcggtaagatccttgagagttttcgccccgaagaacgttttccaatgatgagcacttttaaagttctgctatgtggcgcggtattatcccgtattgacgccgggcaagagcaactcggtcgccgcatacactattctcagaatgacttggttgagtactcaccagtcacagaaaagcatcttacggatggcatgacagtaagagaattatgcagtgctgccataaccatgagtgataacactgcggccaacttacttctgacaacgatcggaggaccgaaggagctaaccgcttttttgcacaacatgggggatcatgtaactcgccttgatcgttgggaaccggagctgaatgaagccataccaaacgacgagcgtgacaccacgatgcctgtagcaatggcaacaacgttgcgcaaactattaactggcgaactacttactctagcttcccggcaacaattaatagactggatggaggcggataaagttgcaggaccacttctgcgctcggcccttccggctggctggtttattgctgataaatctggagccggtgagcgtgggtctcgcggtatcattgcagcactggggccagatggtaagccctcccgtatcgtagttatctacacgacggggagtcaggcaactatggatgaacgaaatagacagatcgctgagataggtgcctcactgattaagcattggtaactgtcagaccaagtttactcatatatactttagattgatttaaaacttcatttttaatttaaaaggatctaggtgaagatcctttttgataatctcatgaccaaaatcccttaacgtgagttttcgttccactgagcgtcagaccccgtagaaaagatcaaaggatcttcttgagatcctttttttctgcgcgtaatctgctgcttgcaaacaaaaaaaccaccgctaccagcggtggtttgtttgccggatcaagagctaccaactctttttccgaaggtaactggcttcagcagagcgcagataccaaatactgttcttctagtgtagccgtagttaggccaccacttcaagaactctgtagcaccgcctacatacctcgctctgctaatcctgttaccagtggctgctgccagtggcgataagtcgtgtcttaccgggttggactcaagacgatagttaccggataaggcgcagcggtcgggctgaacggggggttcgtgcacacagccc

SEQ ID NO: 86 - DNA, 8890 bp, synthetic construct
  source 1..8890: mol_type = other DNA
gcgcagataccaaatactgttcttctagtgtagccgtagttaggccaccacttcaagaactctgtagcaccgcctacatacctcgctctgctaatcctgttaccagtggctgctgccagtggcgataagtcgtgtcttaccgggttggactcaagacgatagttaccggataaggcgcagcggtcgggctgaacggggggttcgtgcacacagcccagcttggagcgaacgacctacaccgaactgagatacctacagcgtgagctatgagaaagcgccacgcttcccgaagggagaaaggcggacaggtatccggtaagcggcagggtcggaacaggagagcgcacgagggagcttccagggggaaacgcctggtatctttatagtcctgtcgggtttcgccacctctgacttgagcgtcgatttttgtgatgctcgtcaggggggcggagcctatggaaaaacgccagcaacgcggcctttttacggttcctggccttttgctggccttttgctcacatgttctttcctgcgttatcccctgattctgtggataaccgtattaccgcctttgagtgagctgataccgctcgccgcagccgaacgaccgagcgcagcgagtcagtgagcgaggaagcagatctgcggccgcactagtgctagactgccatgtcgagggattccgggtcactgtgagtgggggaggcagggaagaagggctcacaggacagtcaaaccatgccccctgtttttccttcttcaagtagacctctataagacaacagagacaactaaggctgagtggccaggcgaggagaaaccatctcgccgtaaaacatggaaggaacacttcaggggaaaggtggtatctctaagcaagagaactgagtggagtcaaggctgagagatgcaggataagcaaatgggtagtgaaaagacattcatgaggacagctaaaacaataagtaatgtaaaatacagcatagcaaaactttaacctccaaatcaagcctctacttgaatccttttctgagggatgaataaggcataggcatcaggggctgttgccaatgtgcattagctgtttgcagcctcaccttctttcatggagtttaagatatagtgtattttcccaaggtttgaactagctcttcatttctttatgttttaaatgcactgacctcccacattccctttttagtaaaatattcagaaataatttaaatacatcattgcaatgaaaataaatgttttttattaggcagaatccagatgctcaaggcccttcataatatcccccagtttagtagttggacttagggaacaaaggaacctttaatagaaattggacagcaagaaagcgagcttagtgatacttgtgggccagggcattagccacaccagccaccactttctgataggcagcctgcactggtggggtgaattccgcggaagcttgtgtaattgttaatttctctgtcccactccatccaggtcgtgtgattccaaatctgttccagagatttattactccaactagcattccaaggcacagcagtggtgcaaatgagttttccagagcaaccccaaatccccaggagctgttgatcctttaggtatctttccacagccaggattcttgcctggagctgcttgatgccccagactgtgagttgcaacagatgctgttgcgcctcaatagccctcagcaaattgttctgctgctgcactataccagacaataattgtctggcctgtaccgtcagcgtcattgacgctgcgcccatagtgcttcctgctgctcccaagaacccaaggaacaaagctcctgcggccgctccggaattccatgtgttaatcctcatcctgtctacttgccacacaatcatcacctgccatctgttttccataatccctgatgatctttgcttttcttcttggcactacttttatgtcactattatcttgtattactactgccccttcacctttccagaggagctttgctggtcctttccaaactggatctctgctgtccctgtaataaacccgaaaattttgaatttttgtaatttgtttttgtaattctttagtttgtatgtctgttgctattatgtctactattctttcccctgcactgtaccccccaatccccccttttcttttaaaattgtggatgaatactgccatttgtactgctgtcttaagatgttcagcctgatctcttacctgtcctataattttctttaattctttattcatagattctattactccttgactttggggattgtagggaatgccaaattcctgcttgatccccgcccaccaacaggcggccttaactgtagtactggtgaaattgctgccattgtctgtatgtactgtttttactggccatcttcctgctaattttaagaggaagtatgctgtttcttgccctgtctctgctggaattacttctgcttctatatatccactggctacatgaactgctaccaagataacttttccttctaaatgtgtacaatctagctgccatattcctgggctacagtctacttgtccatgcatggcttccccttttagctgacatttatcacagctggctactatttcttttgctactacaggtggtaggttaaaatcactagccattgctctccaattactgtgatatttctcatgttcttcttgggccttatctattccatctaaaaatagtactttcctgattccagcactgaccaatttatctacttgttcatttcctccaattcctttgtgtgctggtacccatgccaggtagactttttccttttttattaactgctctattatttgactgactaactctgattcactcttatctggttgtgcttgaatgattcccaatgcatattgtgagtctgtcactatgtttacttctaatcccgaatcctgcaaagctagatgaattgcttgtaactcagtcttctgatttgttgtgtccgttagggggacaactttttgtcttcctctgtcagttacatatcctgcttttcctaatttagtttccctattggctgccccatctacatagaaagtttctgctcctattatgggttctttctctaactggtaccataacttcactaagggaggggtattgacaaactcccactcaggaatccaggtggcttgccaatactctgtccaccatgcttcccatgtttccttttgtatgggtaatttaaatttaggagtctttccccatattactatgctttctgtggctattttttgtactgcctctgttaattgtttcacatcattagtgtgggcacccttcattcttgcatactttcctgttttcagatttttaaatggctcttgataaatttgatatgtccattggccttgcccctgcttctgtatttctgctattaagtcttttgatgggtcataatacactccatgtaccggttcttttagaatctccctgttttctgccagttctagctctgcttcttctgttagtggtactacttctgttagtgctttggttcccctaagaagtttacataattgccttactttaatccctgcataaatctgacttgcccaattcaattttcccactaatttctgtatgtcattgacagtccagctgtccttttctggcagcactataggctgtactgtccatttatcaggatggagttcataacccatccaaaggaatggaggttctttctgatgttttttgtctggtgtggtaaatccccacctcaacagatgttgtctcagttcctctatttttgttctatgctgccctatttctaagtcagatcctacatacaaatcatccatgtattgatagatgactatgtctggattttgttttctaaaaggctctaagatttttgtcatgctacactggaatattgctggtgatcctttccatccctgtggaagcacattgtactgatatctaatccctggtgtctcattgtttatactaggtatggtaaatgcagtatacttcctgaagtctttatctaagggaactgaaaaatatgcatcgcccacatccagtactgttactgattttttctgttttaaccctgcaggatgtggtattcctaattgaacttcccagaaatcttgagttctcttattaagttctctgaaatctactaattttctccatttagtactgtcttttttctttatggcaaatactggagtattgtatggattttcaggcccaatttttgaaatttttccttccttttccatttctgtacaaatttctactaatgcttttattttttcttctgtcaatggccattgtttaacttttgggccatccattcctggctttaattttactggtacagtctcaataggactaatgggaaaatttaaagtgcagccaatctgagtcaacagatttcttccaattatgttgacaggtgtaggtcctactaatactgtacctatagctttatgtccgcagatttctatgagtatctgatcatactgtcttactttgataaaacctccaattccccctatcatttttggtttccatcttcctggcaaattcatttcttctaatactgtatcatctgctcctgtatctaatagagcttcctttaattgcccccctatctttattgtgacgaggggtcgctgccaaagagtgatctgagggaagctaaaggatacagttccttgtctatcggctcctgcttctgagagggagttgttgtctcttccccaaacctgaagctctcttctggtggggctgttggctctggtctgctctgaagaaaattccctggccttcccttgtgggaaggccagatcttccctaaaaaattagcctgtctctcagtacaatctttcatttggtgtccttcctttccacatttccaacagccctttttcctaggggccctgcaatttttggctatgtgcccttctttgccacaattgaaacacttaacagtctttctttggttcctaaaattgcctttctgtatcattatggtagctggatttgttacttggctcattgcttcagccaaaactcttgctttatggccgggtccccccactccctgacatgctgtcatcatttcttctagtgtcgctcctggtcccaatgcttttaaaatagtcttacaatctgggttcgcattttggaccaacaaggtttctgtcatccaattttttacctcttgtgaagcttgctcggctcttagagttttatagaatcggtctacatagtctctaaagggttcctttggtccttgtcttatgtccagaatgctggtagggctatacattcttactattttatttaatcccaggattatccatcttttatagatttctcctactgggataggtggattatgtgtcatccatcctatttgttcctgaagggtactagtagttcctgctatgtcacttccccttggttctctcatctggcctggtgcaataggccctgcatgcactggatgcactctatcccattctgcagcttcctcattgatggtctcttttaacatttgcatggctgcttgatgtccccccactgtgtttagcatggtgtttaaatcttgtggggtggctccttctgataatgctgaaaacatgggtatcacttctgggctgaaagccttctcttctactacttttacccatgcatttaaagttctaggtgatatggcctgatgtaccatttgcccctggatgttctgcactatagggtaattttggctgacctgattgctgtgtcctgtgtcagctgctgcttgctgtgcttttttcttacttttgttttgctcttcctctatcttgtctaaagcttccttggtgtcttttatctctatcctttgatgcacacaatagagggttgctactgtattatataatgatctaagttcttctgatcctgtctgaagggatggttgtagctgtcccagtatttgtctacagccttctgatgtttctaacaggccaggattaactgcgaatcgttctagctccctgcttgcccatactatatgttttaatttatattttttctttccccctggccttaaccgaattttttcccatcgatctaattctcccccgcttaatactgacgctctcgcacccatggcggcggcagatctcgaattcagatctcacgtgctttgccaaagtgatgggccagcacacagaccagcacgttgcccaggagctgtgggaggaagataagaggtatgaacatgattagcaaaagggcctagcttggactcagaataatccagccttatcccaaccataaaataaaagcagaatggtagctggattgtagctgctattagcaatatgaaacctcttacatcagttacaatttatatgcagaaatatttatatgcagaaatattgctattgccttaacccagaaattatcactgttattctttagaatggtgcaaagaggcatgatacattgtatcattattgccctgaaagaaagagattagggaaagtattagaaataagataaacaaaaaagtatattaaaagaagaaagcattttttaaaattacaaatgcaaaattaccctgatttggtcaatatgtgtaccctgttacttctccccttcctatgacatgaacttaaccatagaaaagaaggggaaagaaaacatcaagggtcccatagactcaccctgaagttctcaggatccgagctcggtaccacatgtaagcttcgaggggaggctggatcggtcccggtgtcttctatggaggtcaaaacagcgtggatggcgtctccaggcgatctgacggttcactaaacgagctctgcttatatagacctcccaccgtacacgcctaccgcccatttgcgtcaatggggcggagttgttacgacattttggaaagtcccgttgattttggtgccaaaacaaactcccattgacgtcaatggggtggagacttggaaatccccgtgagtcaaaccgctatccacgcccattgatgtactgccaaaaccgcatcaccatggtaatagcgatgactaatacgtagatgtactgccaagtaggaaagtcccataaggtcatgtactgggcataatgccaggcgggccatttaccgtcattgacgtcaatagggggcgtacttggcatatgatacacttgatgtactgccaagtgggcagtttaccgtaaatactccacccattgacgtcaatggaaagtccctattggcgttactatgggaacatacgtcattattgacgtcaatgggcgggggtcgttgggcggtcagccaggcgggccatttaccgtaagttatgtaacgcggaactccatatatgggctatgaactaatgaccccgtaattgattactattaataactagtcaataatcaatgtcaacatggcggtaatgttggacatgagccaatataaatgtacatattatgatatggatacaacgtatgcaatgggccaagctcatggctgactaattttttttatttatgcagaggccgaggccggatcctctagcccatgggggccccctcaggggatccacgtcaggtggcacttttcggggaaatgtgcgcggaacccctatttgtttatttttctaaatacattcaaatatgtatccgctcatgagacaataaccctgataaatgcttcaataatattgaaaaaggaagagtatgagtattcaacatttccgtgtcgcccttattcccttttttgcggcattttgccttcctgtttttgctcacccagaaacgctggtgaaagtaaaagatgctgaagatcagttgggtgcacgagtgggttacatcgaactggatctcaacagcggtaagatccttgagagttttcgccccgaagaacgttttccaatgatgagcacttttaaagttctgctatgtggcgcggtattatcccgtattgacgccgggcaagagcaactcggtcgccgcatacactattctcagaatgacttggttgagtactcaccagtcacagaaaagcatcttacggatggcatgacagtaagagaattatgcagtgctgccataaccatgagtgataacactgcggccaacttacttctgacaacgatcggaggaccgaaggagctaaccgcttttttgcacaacatgggggatcatgtaactcgccttgatcgttgggaaccggagctgaatgaagccataccaaacgacgagcgtgacaccacgatgcctgtagcaatggcaacaacgttgcgcaaactattaactggcgaactacttactctagcttcccggcaacaattaatagactggatggaggcggataaagttgcaggaccacttctgcgctcggcccttccggctggctggtttattgctgataaatctggagccggtgagcgtgggtctcgcggtatcattgcagcactggggccagatggtaagccctcccgtatcgtagttatctacacgacggggagtcaggcaactatggatgaacgaaatagacagatcgctgagataggtgcctcactgattaagcattggtaactgtcagaccaagtttactcatatatactttagattgatttaaaacttcatttttaatttaaaaggatctaggtgaagatcctttttgataatctcatgaccaaaatcccttaacgtgagttttcgttccactgagcgtcagaccccgtagaaaagatcaaaggatcttcttgagatcctttttttctgcgcgtaatctgctgcttgcaaacaaaaaaaccaccgctaccagcggtggtttgtttgccggatcaagagctaccaactctttttccgaaggtaactggcttcagcaga

SEQ ID NO: 87 - protein, 107 aa, synthetic construct
DIQMTQTTSSLSASLGDRVTISCRASQDISKYLNWYQQKPDGTVKLLIYHTSRLHSGVPSRFSGSGSGTDYSLTISNLEQEDIATYFCQQGNTLPYTFGGGTKLEIT

SEQ ID NO: 88 - protein, 119 aa, synthetic construct [sequence omitted]

SEQ ID NO: 89 - protein, 123 aa, synthetic construct
QVQLVESGGGLVQPGGSLKLSCAASGFDFSRYWMSWVRQAPGKGLEWIGEINPTSSTINFTPSLKDKVFISRDNAKNTLYLQMSKVRSEDTALYYCARGNYYRYGDAMDYWGQGTSVTVSKIS

SEQ ID NO: 90 - protein, 122 aa, synthetic construct
QIQLVQSGPELKKPGETVNISCKASGYTFTNYGMNWVKQAPGKGLKWMGWINTNTGEPKYAEEFKGRFALSLETSASTAYLQINNLKNEDTATYFCARGYGNYARGAWLAYWGQGTLVTVSA

SEQ ID NO: 91 - protein, 121 aa, synthetic construct [sequence omitted]

SEQ ID NO: 92 - protein, 119 aa, synthetic construct
QVQLVESGGGVVQPGRSLRLSCAASGFSFSSYVCWVRQAPGKGLEWIACIYTGDGTNYSASWAKGRFTISKDSSKNTVYLQMNSLRAEDTAVYFCARPDITYGFAINFWGPGTLVTVSS

SEQ ID NO: 93 - protein, 120 aa, synthetic construct
EVQLVESGGGLVQPGRSLRLSCAASGFTFSNYGMAWVRQAPGKGLEWVATISYDGSITYYRDSVKGRFTISRDNSKNTLYLQMNSLRAEDTAVYYCTREEQYSSWYFDFWGQGILVTVSS

SEQ ID NO: 94 - protein, 122 aa, synthetic construct
EVQLQQSGPELVKPGASMKISCKASGYSFTGYTMNWVKQSHGKNLEWMGLINPYKGVSTYNQKFKDKATLTVDKSSSTAYMELLSLTSEDSAVYYCARSGYYGDSDWYFDVWGQGTTLTVFS

SEQ ID NO: 95 - protein, 120 aa, synthetic construct
QVQLKQSGPGLVQPSQSLSLTCTVSGFSLTSYGVHWVRQPPGKGLEWLGVIWSGGSTDYNAAFISRLSIRKDNSKSQVFFKMNSLQADDTAIYYCARTFTTSTSAWFAYWGQGTLVTVSA

SEQ ID NO: 96 - protein, 120 aa, synthetic construct
EVKLQESGPGLVAPSQSLSVTCTVSGVSLPDYGVSWIRQPPRKGLEWLGVIWGSETTYYNSALKSRLTIIKDNSKSQVFLKMNSLQTDDTAIYYCAKHYYYGGSYAMDYWGQGTSVTVSS

SEQ ID NO: 97 - protein, 107 aa, synthetic construct
QIVLTQSPAIMSASPGEKVTMTCSASSSVSYMNWYQQKSGTSPKRWIYDTSKLASGVPAHFRGSGSGTSYSLTISGMEAEDAATYYCQQWSSNPFTFGSGTKLEINR

SEQ ID NO: 98 - protein, 112 aa, synthetic construct
SDIVLTQSPASLAVSLGQRATISCRASKSVSTSGYSYLHWYQQKPGQPPKLLIYLASNLESGVPARFSGSGSGTDFTLNIHPVEEEDAATYYCQHSRELPFTFGSGTKLEIK

SEQ ID NO: 99 - protein, 113 aa, synthetic construct
DVLLTQTPLSLPVSLGDQASISCRSSQTIVHSNGNTYLEWFLQKPGQSPKLLIYQVSNRFSGVPDRFSGSGSGTDFTLKISRVEAEDLGVYYCFQGSHVPRTFGGGTKLEIKR

SEQ ID NO: 100 - protein, 107 aa, synthetic construct
QIVLSQSPAILSASPGEKVTMTCRASSSVSYIHWFQQKPGSSPKPWIYATSNLASGVPVRFSGSGSGTSYSLTISRVEAEDAATYYCQQWTSNPPTFGGGTKLEIKR

SEQ ID NO: 101 - protein, 130 aa, synthetic construct
MDMRVPAQLLGLLLLWLRGARCDIQMTQSPSSLSASVGDRVTIKCQASQSISSRLAWYQQKPGKPPKLLIYRASTLASGVPSRFSGSGSGTDFTLTISSLQPEDVATYYCQCTGYGISWPIGGGTKVEIK

SEQ ID NO: 102 - protein, 111 aa, synthetic construct
DIQLTQSPSSLSASVGDRVTITCRASQSVSISSHDLMQWYQQKPGKAPKLLIYDAFNLASGVPSRFSGSGSGTDFTLTISSLQPEDFATYYCQQSKDDPYTFGQGTKLEIK

SEQ ID NO: 103 - protein, 108 aa, synthetic construct
MDIQMTQTTSSLSASLGDRVTISCRASQDIRNYLNWYQQKPDGTVKLLIYYTSRLHSGVPSKFSGSGSGTDYSLTISNLEQEDIATYFCQQGNTLPWTFAGGTKLEIK

SEQ ID NO: 104 - protein, 108 aa, synthetic construct
SIVMTQTPKFLLVSAGDRVTITCKASQSVSNDVAWYQQKPGQSPKLLIYYASNRYTGVPDRFTGSGYGTDFTFTISTVQAEDLAVYFCQQDYSSPPWTFGGGTKLEIR

SEQ ID NO: 105 - DNA, 438 bp, synthetic construct
  source 1..438: mol_type = other DNA
ggtgatcagaatcctcaaattgcggcacatgtcataagtgaggccagcagtaaaacaacatctgtgttacagtgggctgaaaaaggatactacaccatgagcaacaacttggtaaccctggaaaatgggaaacagctgaccgttaaaagacaaggactctattatatctatgcccaagtcaccttctgttccaatcgggaagcttcgagtcaagctccatttatagccagcctctgcctaaagtcccccggtagattcgagagaatcttactcagagctgcaaatacccacagttccgccaaaccttgcgggcaacaatccattcacttgggaggagtatttgaattgcaaccaggtgcttcggtgtttgtcaatgtgactgatccaagccaagtgagccatggcactggcttcacgtcctttggcttactcaaactc

SEQ ID NO: 106 - protein, 146 aa, synthetic construct
GDQNPQIAAHVISEASSKTTSVLQWAEKGYYTMSNNLVTLENGKQLTVKRQGLYYIYAQVTFCSNREASSQAPFIASLCLKSPGRFERILLRAANTHSSAKPCGQQSIHLGGVFELQPGASVFVNVTDPSQVSHGTGFTSFGLLKL

SEQ ID NO: 107 - protein, 123 aa, synthetic construct; identical to SEQ ID NO: 89

SEQ ID NO: 108 - protein, 112 aa, synthetic construct; identical to SEQ ID NO: 98